European Patent Application EP 4 470 364 A1, published December 4, 2024. Title: TOMATO CONTAINING HIGH CONCENTRATION OF 7-DEHYDROCHOLESTEROL AND METHOD FOR PRODUCING THE SAME. Applicant: (주)지플러스생명과학. The sequence listing filed with the application follows.

SEQUENCE LISTING (78 sequences)

SEQ ID NO: 1 - DNA, 1678 bp, synthetic construct
  misc_feature 1..1678: note = nucleotides coding DWF5 of S. lycopersicum
  source 1..1678: mol_type = other DNA
ttagtcagtacaacagatttttataattgagagaatctgagaagaggacctataccactgtggagagagtggagtaaacacagagcactaaaaatcagtgaattaaagtctacatataagtcaagattccatattgggcggagacttctgtagttccagtttttttcttcaaaaccccaaaatcagcaaaagctgaattgattgaggaagaagaagaagaagaaaaaatggtggagaacaagttggtacactctccattaatcacttatggatcaatgctcagtcttctatctttcacaccaccttttgtaatcctcatgtggtatacaaatgtgcacgctgatgggtctatcttgaaaacgttcaatcatctaagggaaaatggtttgcaaggattaattgatatttggccaaaacctactgcaattgctgggaagctaatcatttgttatgctctatttgaggcggcactacagcttctattgcctggtaaaacagtcgaaggcccaatatctccaactggacataggcctgtctataaggctaatggcatggcagcatatgcagtgacactgatcacatatatcagtctctggtggtttggaatatttaatcctgcaattgtttatgaccatctgggcgagattttctctacacttatttttgggagtttagtcttctgtgttttattgtacattaaaggtcatgttgcaccatcttccactgattccggctcatcagggaacataatagttgacttctattggggtatggagctttatcctcgtatcgggaaacacttcgatattaaagtcttcacaaactgcagatttggtatgatgtcttgggcagttcttgctgtcacgtattgcataaaacagcatgaagaatatgggcgtgtatctgattccatgcttgtaaatacgatattgatgttggtgtatgtcacaaaattcttttggtgggaagctgggtactggaacacaatggatattgcacatgacagagctggcttttatatatgttggggatgcttggtgtgggttccaagcatatatacgtctcctggaatgtatcttgttaaacaacctgtgaatcttgggcttcagctttccctttacatactagtggctggtcttctctgcatatatatcaactatgattgtgacaggcagaggcaagagttccggagaacaaatggaaaatgcactgtctggggaaagactccatctaagatagtcgccgcatacactactacctctggtgagaaaaagaccagccttctgcttacatcaggatggtggggcttagctcgccatttccactatgttccagaaatattagcggcatttttctggagtgtaccagctcttttcaaccacttcattccctacttctacgtcatctttctaataatcctccttctcgatcgagctaaaagggacgatgaccgatgcaaggcaaagtatggcaagtactggaaattgtattgtgaaaaggttccttacagagttatcccaggaatttactagtgatttttggacttctaagaatgttttactataaagtttgatgtattttgtagcctcttcatgttgttgtttgtatgtacacttattagttccaacagttttgagaaacttgtttttatataaaaatagtgaagacgcgagttgag

SEQ ID NO: 2 - protein, 434 aa, synthetic construct
  REGION 1..434: note = DWF5 of S. lycopersicum
MVENKLVHSPLITYGSMLSLLSFTPPFVILMWYTNVHADGSILKTFNHLRENGLQGLIDIWPKPTAIAGKLIICYALFEAALQLLLPGKTVEGPISPTGHRPVYKANGMAAYAVTLITYISLWWFGIFNPAIVYDHLGEIFSTLIFGSLVFCVLLYIKGHVAPSSTDSGSSGNIIVDFYWGMELYPRIGKHFDIKVFTNCRFGMMSWAVLAVTYCIKQHEEYGRVSDSMLVNTILMLVYVTKFFWWEAGYWNTMDIAHDRAGFYICWGCLVWVPSIYTSPGMYLVKQPVNLGLQLSLYILVAGLLCIYINYDCDRQRQEFRRTNGKCTVWGKTPSKIVAAYTTTSGEKKTSLLLTSGWWGLARHFHYVPEILAAFFWSVPALFNHFIPYFYVIFLIILLLDRAKRDDDRCKAKYGKYWKLYCEKVPYRVIPGIY

SEQ ID NO: 3 - DNA, 1735 bp, synthetic construct
  misc_feature 1..1735: note = nucleotides coding DWF5 of S. lycopersicum
  source 1..1735: mol_type = other DNA
tagaagaatcagcggagagttggagaaccacgttagcagtatacgacaaggaagattaccagtgtccagtgtgcgtgtgtgtaatttataatcaacaaaattagcagtggccgagttatcttttagtttttcaaaaacaagaagaggtgcagagaacagggagggaggaagaagcaatggcggagtctcagttggttcaccctcctttattcacctatatctcaatgatcactctgctcactttagtacccccttttgttattctcatgtggtatacaaatgttcatgctgatggatctgtattgcaaacatataattatctaaaggagaatggcctgcaaggactaattgacatttggccaagacccactgcaattgcgggaaaaataataatttgctatgctctatttgaggctacacttcagcttttgttgcctggtaaaagggttgaaggaccgatatctcctactggacacaggcctgtctataaggcaaatggcatggcagcatatacagtgacactaattacctatctcagcctttggtggtttggaatattcaatcctacaatcgtgtatgatcatctgggagagattctctctacactaaattttggaagcttaatcttctgtctctttttatacataaaaggtcatgttgcaccatcttccactgatcacggttcatcagggaacataatagttgactactattgggggatggagttgtatcctcgcattggcaaacactttgatatcaaggtcttcacaaactgcagatttggcatgatatcttggggactcctccctattacctactgtataaagcagtatgaagaatatggaagtctctctgattccatgcttatacataccataataacgttggtgtatgtcacgaaattcttttggtgggaagcaggttactggaacaccatggatattgctcatgacagagccggtttttacatatgctggggttgcttggtatttcttccatgtatgtacacttctcctggcatgtaccttgtcaaacatcctgtaaatcttggacctcagcttgcaatttctatcctagtagctggtattctctgcgtatacataaactatgattgtgacagacagaggcaagagttccgcagaacaaatggcaaagcccttgtctggggaaaggctccttcaaagattgtcgcctcatacactactacaactggcgaaactaaaaccagcattctcctgacatctggatggtggggcttatcgcggcatttccattatgttccagaaatactagcttcgtttttctggagtgtgccagctcttctcaaccatttcatgccctacatctatgtaatctatctgacgggcctccttttggatcgagccaaaagggatgacgaaaggtgcaagtcaaagtatggcaaatactggaaaaagtattgtgaaaaggtgccttaccgggtagtccctggaatttattagtgattcttgagcttcaactgatgaactgtctttaatagtgctgcttctagtattgtagtagtatttagaccatgaaaaattttcttctttcaataaagcacttttagttgaaccaacatctcatttctatggttgtaagttgttacacgatgaaaaaatcagcttgaaatagatatgccgtgaaattagttgaggtgtgtgaaaactcggaccagtttgaaatattgttccaattaaaatgaacactaaaacag

SEQ ID NO: 4 - protein, 434 aa, synthetic construct
  REGION 1..434: note = DWF5 of S. lycopersicum
MAESQLVHPPLFTYISMITLLTLVPPFVILMWYTNVHADGSVLQTYNYLKENGLQGLIDIWPRPTAIAGKIIICYALFEATLQLLLPGKRVEGPISPTGHRPVYKANGMAAYTVTLITYLSLWWFGIFNPTIVYDHLGEILSTLNFGSLIFCLFLYIKGHVAPSSTDHGSSGNIIVDYYWGMELYPRIGKHFDIKVFTNCRFGMISWGLLPITYCIKQYEEYGSLSDSMLIHTIITLVYVTKFFWWEAGYWNTMDIAHDRAGFYICWGCLVFLPCMYTSPGMYLVKHPVNLGPQLAISILVAGILCVYINYDCDRQRQEFRRTNGKALVWGKAPSKIVASYTTTTGETKTSILLTSGWWGLSRHFHYVPEILASFFWSVPALLNHFMPYIYVIYLTGLLLDRAKRDDERCKSKYGKYWKKYCEKVPYRVVPGIY

SEQ ID NO: 5 - DNA, 1742 bp, synthetic construct
  misc_feature 1..1742: note = nucleotides coding CPD of S. lycopersicum
  source 1..1742: mol_type = other DNA
gcagagcgttttgcatacaaaaaaaaattaattaacatggataccatcgatctttttctctatctttttctctctgttttcaccttttatctcctccggtgtatggcggcggcccatcttcgcgggcgtaaaactcgactcccgccgggaacccttggcctcccgtttatcggagaaaccctccagttaatttctgcgtacaaaacggaaaatcctgaaccgttcatcgatgaccgtgtttcaaaatacggcagcattttcacgacccatgtttttggtgaaccgacggttttctctgctgacccggaaacgaaccggtttattttgcagaatgaaggtcggctttttgagtcgagttatcccggttcgatacagaatttacttgggagatactctctgttgcttatgagaggaagtctacacaaacgaatgcattcattaactatgagttttgctaattcttccattcttaaagatcatctgttgggcgatatagatcgattggttaggcttaatttggattcatggaccggcagggttttcctcatggacgaggctaagaagataacgtttaatctaacagtgaagcagttgatgagttttgatccatgtgagtggacagagaatctgatgaaagagtatatgcttgttattgaaggtttcttctgcattcctttgcctattttctcatccacctatcgcaaggccattcaagcgagaacgaaagtagcggaggcgttgggattggtagtgagagatcggagaaaagaacgagacggaggagaacgaaagaatgatatgttggaggcattgttcgaaggagacggagttgaaggagtaggattttccgatgaggaaattgttgattttatactggcgttgcttgttgctggctatgaaactacctccaccatcatgacccttgctgtaaaattcctcacggagacaccccgtgctctatcactacttaaggaagagcacgaggagatcaggttaagaaaaggtgaagttaagtctttacaatgggaagattacaagtcaatgcccttcactcaatgcgttgttaatgaaactctgcgaatcgctaacataattagtggagtgttcaggagagccatgactgacataaatatcaaaggttataccattccaaaaggttggaaggtttttgcttctctccgagctgttcatctagaccatgaacatttcaaagatgcgcgtacatttgatccatggaggtggcagagtagtgcaggaccgacaagctcacctaacgtattcacaccatttggtggtggacctcgtcgatgtcctggttacgagcttgctagagtggaactctctgttttccttcaccacttggtgactcgttttagttgggttccggctgaggcagataagttagttttcttcccaacgacaaggatgctgaagcgatatccaattaacgtccaacatcgaagcttgtttgagcagaaagaagaagagaagggttcgtgagattgtagaatgcagagtggagggaggtgtatgaaaggtgttaaataagacaatagtatataggtgttagcatatacttagaaaattaaattatttgtagtgaattgagcagagattaacattcctctgatctgcaaggggaatcaggaagattttattctgagcaattggttattatataatagtaatgcacagtttttaatgtatgttaattagcatgattaaagatttaattgccctca

SEQ ID NO: 6 - protein, 487 aa, synthetic construct
  REGION 1..487: note = CPD of S. lycopersicum
MDTIDLFLYLFLSVFTFYLLRCMAAAHLRGRKTRLPPGTLGLPFIGETLQLISAYKTENPEPFIDDRVSKYGSIFTTHVFGEPTVFSADPETNRFILQNEGRLFESSYPGSIQNLLGRYSLLLMRGSLHKRMHSLTMSFANSSILKDHLLGDIDRLVRLNLDSWTGRVFLMDEAKKITFNLTVKQLMSFDPCEWTENLMKEYMLVIEGFFCIPLPIFSSTYRKAIQARTKVAEALGLVVRDRRKERDGGERKNDMLEALFEGDGVEGVGFSDEEIVDFILALLVAGYETTSTIMTLAVKFLTETPRALSLLKEEHEEIRLRKGEVKSLQWEDYKSMPFTQCVVNETLRIANIISGVFRRAMTDINIKGYTIPKGWKVFASLRAVHLDHEHFKDARTFDPWRWQSSAGPTSSPNVFTPFGGGPRRCPGYELARVELSVFLHHLVTRFSWVPAEADKLVFFPTTRMLKRYPINVQHRSLFEQKEEEKGS

SEQ ID NO: 7 - DNA, 1782 bp, synthetic construct
  misc_feature 1..1782: note = nucleotides coding SMT1 of S. lycopersicum
  source 1..1782: mol_type = other DNA
tagggggtgaaggagacgtggtataatatgtgacgtggccacgaacccccacttctgtttatggtgtctttcaatttttgagtgctggcattaggcgtatatatatatatgagttgttgctgtagttgtttacagcatatttgctttttctaaggatccgtctccgttttggcatttccttttccgtttttttccatcttaaagttgtaagctttctacttttctttttttcttctgcattgttaatctttacttgatttcatcatggggtttgtttaatcttgtttatagatcttgtgatttgggaaaagagatgtcaaaacaaggggcttttgatctggcatttggggttggaggaagaattggcaaggatgaagttctctctgctgttgacaaatatgagaagtaccatggttattatggaggtgaagaagacgagagaaagaataactacactgacatggtaaacaaatactatgatctttgcaccagcttctatgaatacggatggggagagtccttccattttgcgcccagatggaaagaagaatcactccaggaaagcattaagaggcatgagcacttccttgccttgcaactgggattgaaaccaggacaaaaggtcttggatgtaggatgtggaattggagggccgttaagagaaattgctcgattcagctctacatcagttacaggcctcaacaacaatgaatatcagatatctcgaggacaggtgttgaaccgcaaagtgggattggatcaaacttgcaactttgtaaagggtgatttcatgaaaatgccattccctgacaatagctttgatgcagtatatgcaatagaagctacctgccatgcaccagatccggttggatgctatagagagatctatagggtgctgaagcctggtcagtgctttgctgtgtatgagtggtgcatgactgatgcatacaatccaaataatgaagagcagaaaagaatcaaggaagaaattgagctcggaaatggtctcccggagattagatcaacacaacagtgcctagaagcagcgagaaaagctggttttgaagttgtgtgggataaggatctcgctgaagactcaccagtttcatggtacatgcctttagatacaagtcacttctcactcagtagcttccgcctaacagcagttggcagacttttcaccagaaatctggtttcggcacttgaatatgtgggtgtagctcctaaaggtagtcaaagggttcaagctttcttagaaaaagccgcagaaggtcttgttggtggtgccaagtaagataacaactctacttcatacatacatattagtagagtatcgaacgttataatgatacattaactttttaaacctgtcgttgtcctttcaggaaagggatcttcacaccgatgtatttcttcttggttcgcaagccaatttcagactcacagtaatatttgacttagctcttcattgctttagttagcaaatctttgagattcttggccttgaacttatatggccaggctaatcaaaggttatttcgattttcgtttagggattgggggctatttgtttttcttgcattgcttgtttgtcaccatttttgccatttattgttcttctcaactcctaattgtttgctattttgccattgaattgattgttgtcctggaaaatatgttgttgataaaggtcagcattttgctaaatatatgactaatgacattatggtgatacatcttcttcttcttcttgagagttgataaatattaattattatgtca

SEQ ID NO: 8 - protein, 326 aa, synthetic construct
  REGION 1..326: note = SMT1 of S. lycopersicum
MSKQGAFDLAFGVGGRIGKDEVLSAVDKYEKYHGYYGGEEDERKNNYTDMVNKYYDLCTSFYEYGWGESFHFAPRWKEESLQESIKRHEHFLALQLGLKPGQKVLDVGCGIGGPLREIARFSSTSVTGLNNNEYQISRGQVLNRKVGLDQTCNFVKGDFMKMPFPDNSFDAVYAIEATCHAPDPVGCYREIYRVLKPGQCFAVYEWCMTDAYNPNNEEQKRIKEEIELGNGLPEIRSTQQCLEAARKAGFEVVWDKDLAEDSPVSWYMPLDTSHFSLSSFRLTAVGRLFTRNLVSALEYVGVAPKGSQRVQAFLEKAAEGLVGGAK

SEQ ID NO: 9 - DNA, 114 bp, synthetic construct
  misc_feature 1..114: note = nucleotides coding exon 6 of DWF5 of S. lycopersicum
  source 1..114: mol_type = other DNA
ggtatggagctttatcctcgtatcgggaaacacttcgatattaaagtcttcacaaactgcagatttggtatgatgtcttgggcagttcttgctgtcacgtattgcataaaacag

SEQ ID NO: 10 - DNA, 127 bp, synthetic construct
  misc_feature 1..127: note = nucleotides coding exon 7 of DWF5 of S. lycopersicum
  source 1..127: mol_type = other DNA
catgaagaatatgggcgtgtatctgattccatgcttgtaaatacgatattgatgttggtgtatgtcacaaaattcttttggtgggaagctgggtactggaacacaatggatattgcacatgacagag

SEQ ID NO: 11 - DNA, 126 bp, synthetic construct
  misc_feature 1..126: note = nucleotides coding exon 9 of DWF5 of S. lycopersicum
  source 1..126: mol_type = other DNA
ctttccctttacatactagtggctggtcttctctgcatatatatcaactatgattgtgacaggcagaggcaagagttccggagaacaaatggaaaatgcactgtctggggaaagactccatctaag

SEQ ID NO: 12 - DNA, 65 bp, synthetic construct
  misc_feature 1..65: note = nucleotides coding exon 10 of DWF5 of S. lycopersicum
  source 1..65: mol_type = other DNA
atagtcgccgcatacactactacctctggtgagaaaaagaccagccttctgcttacatcaggatg

SEQ ID NO: 13 - DNA, 82 bp, synthetic construct
  misc_feature 1..82: note = nucleotides coding exon 11 of DWF5 of S. lycopersicum
  source 1..82: mol_type = other DNA
gtggggcttagctcgccatttccactatgttccagaaatattagcggcatttttctggagtgtaccagctcttttcaaccac

SEQ ID NO: 14 - DNA, 131 bp, synthetic construct
  misc_feature 1..131: note = nucleotides coding exon 7 of CPD of S. lycopersicum
  source 1..131: mol_type = other DNA
agtagtgcaggaccgacaagctcacctaacgtattcacaccatttggtggtggacctcgtcgatgtcctggttacgagcttgctagagtggaactctctgttttccttcaccacttggtgactcgttttag

SEQ ID NO: 15 - DNA, 255 bp, synthetic construct
  misc_feature 1..255: note = nucleotides coding exon 8 of CPD of S. lycopersicum
  source 1..255: mol_type = other DNA
ttgggttccggctgaggcagataagttagttttcttcccaacgacaaggatgctgaagcgatatccaattaacgtccaacatcgaagcttgtttgagcagaaagaagaagagaagggttcgtgagattgtagaatgcagagtggagggaggtgtatgaaaggtgttaaataagacaatagtatataggtgttagcatatacttagaaaattaaattatttgtagtgaattgagcagagattaacattcctctgat

SEQ ID NO: 16 - DNA, 48 bp, synthetic construct
  misc_feature 1..48: note = nucleotides coding exon 7 of SMT1 of S. lycopersicum
  source 1..48: mol_type = other DNA
gtgttgaaccgcaaagtgggattggatcaaacttgcaactttgtaaag

SEQ ID NO: 17 - DNA, 117 bp, synthetic construct
  misc_feature 1..117: note = nucleotides coding exon 8 of SMT1 of S. lycopersicum
  source 1..117: mol_type = other DNA
gttggatgctatagagagatctatagggtgctgaagcctggtcagtgctttgctgtgtatgagtggtgcatgactgatgcatacaatccaaataatgaagagcagaaaagaatcaag

SEQ ID NO: 18 - DNA, 126 bp, synthetic construct
  misc_feature 1..126: note = nucleotides coding exon 11 of SMT1 of S. lycopersicum
  source 1..126: mol_type = other DNA
gttgtgtgggataaggatctcgctgaagactcaccagtttcatggtacatgcctttagatacaagtcacttctcactcagtagcttccgcctaacagcagttggcagacttttcaccagaaatctg

SEQ ID NO: 19 - DNA, 98 bp, synthetic construct
  misc_feature 1..98: note = nucleotides coding exon 12 of SMT1 of S. lycopersicum
  source 1..98: mol_type = other DNA
gtttcggcacttgaatatgtgggtgtagctcctaaaggtagtcaaagggttcaagctttcttagaaaaagccgcagaaggtcttgttggtggtgccaa

SEQ ID NO: 20 - DNA, 23 bp, synthetic construct
  misc_feature 1..23: note = D5-1 sgRNA
  source 1..23: mol_type = other DNA
tggagctttatcctcgtatcggg

SEQ ID NO: 21 - DNA, 23 bp, synthetic construct
  misc_feature 1..23: note = D5-2 sgRNA
  source 1..23: mol_type = other DNA
gcagatttggtatgatgtcttgg

SEQ ID NO: 22 - DNA, 23 bp, synthetic construct
  misc_feature 1..23: note = D5-3 sgRNA
  source 1..23: mol_type = other DNA
tgtaaatacgatattgatgttgg

SEQ ID NO: 23 - DNA, 23 bp, synthetic construct
  misc_feature 1..23: note = D5-4 sgRNA
  source 1..23: mol_type = other DNA
gaccagccactagtatgtaaagg

SEQ ID NO: 24 - DNA, 23 bp, synthetic construct
  misc_feature 1..23: note = D5-5 sgRNA
  source 1..23: mol_type = other DNA
tgcattttccatttgttctccgg

SEQ ID NO: 25 - DNA, 23 bp, synthetic construct
  misc_feature 1..23: note = D5-6 sgRNA
  source 1..23: mol_type = other DNA
cctctggtgagaaaaagaccagc

SEQ ID NO: 26 - DNA, 23 bp, synthetic construct
  misc_feature 1..23: note = D5-7 sgRNA
  source 1..23: mol_type = other DNA
agaaagatgacgtagaagtaggg

SEQ ID NO: 27 - DNA, 23 bp, synthetic construct
  misc_feature 1..23: note = C1 sgRNA
  source 1..23: mol_type = other DNA
aacgagtcaccaagtggtgaagg

SEQ ID NO: 28 - DNA, 23 bp, synthetic construct
  misc_feature 1..23: note = C2 sgRNA
  source 1..23: mol_type = other DNA
cgcttcagcatccttgtcgttgg

SEQ ID NO: 29 - DNA, 23 bp, synthetic construct
  misc_feature 1..23: note = C3 sgRNA
  source 1..23: mol_type = other DNA
tgagcagaaagaagaagagaagg

SEQ ID NO: 30 - DNA, 23 bp, synthetic construct
  misc_feature 1..23: note = C4 sgRNA
  source 1..23: mol_type = other DNA
tgagattgtagaatgcagagtgg

SEQ ID NO: 31 - DNA, 23 bp, synthetic construct
  misc_feature 1..23: note = C5 sgRNA
  source 1..23: mol_type = other DNA
gtagaatgcagagtggagggagg

SEQ ID NO: 32 - DNA, 23 bp, synthetic construct
  misc_feature 1..23: note = S1 sgRNA
  source 1..23: mol_type = other DNA
gttgaaccgcaaagtgggattgg

SEQ ID NO: 33 - DNA, 23 bp, synthetic construct
  misc_feature 1..23: note = S2 sgRNA
  source 1..23: mol_type = other DNA
gatgctatagagagatctatagg

SEQ ID NO: 34 - DNA, 23 bp, synthetic construct
  misc_feature 1..23: note = S4 sgRNA
  source 1..23: mol_type = other DNA
gtttcggcacttgaatatgtggg

SEQ ID NO: 35 - DNA, 23 bp, synthetic construct
  misc_feature 1..23: note = S5 sgRNA
  source 1..23: mol_type = other DNA
gccgcagaaggtcttgttggtgg

SEQ ID NO: 36 - DNA, 15954 bp, synthetic construct
  misc_feature 1..15954: note = nucleotides coding D100
  source 1..15954: mol_type = other DNA
aagcttgataatttatttgaaaattcataagaaaagcaaacgttacatgaattgatgaaacaatacaaagacagataaagccacgcacatttaggatattggccgagattactgaatattgagtaagatcacggaatttctgacaggagcatgtcttcaattcagcccaaatggcagttgaaatactcaaaccgccccatatgcaggagcggatcattcattgtttgtttggttgcctttgccaacatgggagtccaagattctgcagtcaaatctcggtgacgggcaggaccggacggggcggtaccggcaggctgaagtccagctgccagaaacccacgtcatgccagttcccgtgcttgaagccggccgcccgcagcatgccgcggggggcatatccgagcgcctcgtgcatgcgcacgctcgggtcgttgggcagcccgatgacagcgaccacgctcttgaagccctgtgcctccagggacttcagcaggtgggtgtagagcgtggagcccagtcccgtccgctggtggcggggggagacgtacacggtcgactcggccgtccagtcgtaggcgttgcgtgccttccaggggcccgcgtaggcgatgccggcgacctcgccgtccacctcggcgacgagccagggatagcgctcccgcagacggacgaggtcgtccgtccactcctgcggttcctgcggctcggtacggaagttgaccgtgcttgtctcgatgtagtggttgacgatggtgcagaccgccggcatgtccgcctcggtggcacggcggatgtcggccgggcgtcgttctgggctcatcgattcgatttggtgtatcgagattggttatgaaattcagatgctagtgtaatgtattggtaatttgggaagatataataggaagcaaggctatttatccatttctgaaaaggcgaaatggcgtcaccgcgagcgtcacgcgcattccgttcttgctgtaaagcgttgtttggtacacttttgactagcgaggcttggcgtgtcagcgtatctattcaaaagtcgttaatggctgcggatcaagaaaaagttggaatagaaacagaatacccgcgaaattcaggcccggttgccatgtcctacacgccgaaataaacgaccaaattagtagaaaaataaaaactgactcggatacttacgtcacgtcttgcgcactgatttgaaaaatctcagccatggctgcaggtcgacgagtcagtaataaacggcgtcaaagtggttgcagccggcacacacgagtcgtgtttatcaactcaaagcacaaatacttttcctcaacctaaaaataaggcaattagccaaaaacaactttgcgtgtaaacaacgctcaatacacgtgtcattttattattagctattgcttcaccgccttagctttctcgtgacctagtcgtcctcgtcttttcttcttcttcttctataaaacaatacccaaagagctcttcttcttcacaattcagatttcaatttctcaaaatcttaaaaactttctctcaattctctctaccgtgatcaaggtaaatttctgtgttccttattctctcaaaatcttcgattttgttttcgttcgatcccaatttcgtatatgttctttggtttagattctgttaatcttagatcgaagacgattttctgggtttgatcgttagatatcatcttaattctcgattagggtttcatagatatcatccgatttgttcaaataatttgagttttgtcgaataattactcttcgatttgtgatttctatctagatctggtgttagtttctagtttgtgcgatcgaatttgtcgattaatctgagtttttctgattaacagccatggactataaggaccacgacggagactacaaggatcatgatattgattacaaagacgatgacgataagatggccccaaagaagaagcggaaggtcggtatccacggagtcccagcagccgacaagaagtacagcatcggcctggacatcggcaccaactctgtgggctgggccgtgatcaccgacgagtacaaggtgcccagcaagaaattcaaggtgctgggcaacaccgaccggcacagcatcaagaagaacctgatcggagccctgctgttcgacagcggcgaaacagccgaggccacccggctgaagagaaccgccagaagaagatacaccagacggaagaaccggatctgctatctgcaagagatcttcagcaacgagatggccaaggtggacgacagcttcttccacagactggaagagtccttcctggtggaagaggataagaagcacgagcggcaccccatcttcggcaacatcgtggacgaggtggcctaccacgagaagtaccccaccatctaccacctgagaaagaaactggtggacagcaccgacaaggccgacctgcggctgatctatctggccctggcccacatgatcaagttccggggccacttcctgatcgagggcgacctgaaccccgacaacagcgacgtggacaagctgttcatccagctggtgcagacctacaaccagctgttcgaggaaaaccccatcaacgccagcggcgtggacgccaaggccatcctgtctgccagactgagcaagagcagacggctggaaaatctgatcgcccagctgcccggcgagaagaagaatggcctgttcggaaacctgattgccctgagcctgggcctgacccccaacttcaagagcaacttcgacctggccgaggatgccaaactgcagctgagcaaggacacctacgacgacgacctggacaacctgctggcccagatcggcgaccagtacgccgacctgtttctggccgccaagaacctgtccgacgccatcctgctgagcgacatcctgagagtgaacaccgagatcaccaaggcccccctgagcgcctctatgatcaagagatacgacgagcaccaccaggacctgaccctgctgaaagctctcgtgcggcagcagctgcctgagaagtacaaagagattttcttcgaccagagcaagaacggctacgccggctacattgacggcggagccagccaggaagagttctacaagttcatcaagcccatcctggaaaagatggacggcaccgaggaactgctcgtgaagctgaacagagaggacctgctgcggaagcagcggaccttcgacaacggcagcatcccccaccagatccacctgggagagctgcacgccattctgcggcggcaggaagatttttacccattcctgaaggacaaccgggaaaagatcgagaagatcctgaccttccgcatcccctactacgtgggccctctggccaggggaaacagcagattcgcctggatgaccagaaagagcgaggaaaccatcaccccctggaacttcgaggaagtggtggacaagggcgcttccgcccagagcttcatcgagcggatgaccaacttcgataagaacctgcccaacgagaaggtgctgcccaagcacagcctgctgtacgagtacttcaccgtgtataacgagctgaccaaagtgaaatacgtgaccgagggaatgagaaagcccgccttcctgagcggcgagcagaaaaaggccatcgtggacctgctgttcaagaccaaccggaaagtgaccgtgaagcagctgaaagaggactacttcaagaaaatcgagtgcttcgactccgtggaaatctccggcgtggaagatcggttcaacgcctccctgggcacataccacgatctgctgaaaattatcaaggacaaggacttcctggacaatgaggaaaacgaggacattctggaagatatcgtgctgaccctgacactgtttgaggacagagagatgatcgaggaacggctgaaaacctatgcccacctgttcgacgacaaagtgatgaagcagctgaagcggcggagatacaccggctggggcaggctgagccggaagctgatcaacggcatccgggacaagcagtccggcaagacaatcctggatttcctgaagtccgacggcttcgccaacagaaacttcatgcagctgatccacgacgacagcctgacctttaaagaggacatccagaaagcccaggtgtccggccagggcgatagcctgcacgagcacattgccaatctggccggcagccccgccattaagaagggcatcctgcagacagtgaaggtggtggacgagctcgtgaaagtgatgggccggcacaagcccgagaacatcgtgatcgaaatggccagagagaaccagaccacccagaagggacagaagaacagccgcgagagaatgaagcggatcgaagagggcatcaaagagctgggcagccagatcctgaaagaacaccccgtggaaaacacccagctgcagaacgagaagctgtacctgtactacctgcagaatgggcgggatatgtacgtggaccaggaactggacatcaaccggctgtccgactacgatgtggaccatatcgtgcctcagagctttctgaaggacgactccatcgacaacaaggtgctgaccagaagcgacaagaaccggggcaagagcgacaacgtgccctccgaagaggtcgtgaagaagatgaagaactactggcggcagctgctgaacgccaagctgattacccagagaaagttcgacaatctgaccaaggccgagagaggcggcctgagcgaactggataaggccggcttcatcaagagacagctggtggaaacccggcagatcacaaagcacgtggcacagatcctggactcccggatgaacactaagtacgacgagaatgacaagctgatccgggaagtgaaagtgatcaccctgaagtccaagctggtgtccgatttccggaaggatttccagttttacaaagtgcgcgagatcaacaactaccaccacgcccacgacgcctacctgaacgccgtcgtgggaaccgccctgatcaaaaagtaccctaagctggaaagcgagttcgtgtacggcgactacaaggtgtacgacgtgcggaagatgatcgccaagagcgagcaggaaatcggcaaggctaccgccaagtacttcttctacagcaacatcatgaactttttcaagaccgagattaccctggccaacggcgagatccggaagcggcctctgatcgagacaaacggcgaaaccggggagatcgtgtgggataagggccgggattttgccaccgtgcggaaagtgctgagcatgccccaagtgaatatcgtgaaaaagaccgaggtgcagacaggcggcttcagcaaagagtctatcctgcccaagaggaacagcgataagctgatcgccagaaagaaggactgggaccctaagaagtacggcggcttcgacagccccaccgtggcctattctgtgctggtggtggccaaagtggaaaagggcaagtccaagaaactgaagagtgtgaaagagctgctggggatcaccatcatggaaagaagcagcttcgagaagaatcccatcgactttctggaagccaagggctacaaagaagtgaaaaaggacctgatcatcaagctgcctaagtactccctgttcgagctggaaaacggccggaagagaatgctggcctctgccggcgaactgcagaagggaaacgaactggccctgccctccaaatatgtgaacttcctgtacctggccagccactatgagaagctgaagggctcccccgaggataatgagcagaaacagctgtttgtggaacagcacaagcactacctggacgagatcatcgagcagatcagcgagttctccaagagagtgatcctggccgacgctaatctggacaaagtgctgtccgcctacaacaagcaccgggataagcccatcagagagcaggccgagaatatcatccacctgtttaccctgaccaatctgggagcccctgccgccttcaagtactttgacaccaccatcgaccggaagaggtacaccagcaccaaagaggtgctggacgccaccctgatccaccagagcatcaccggcctgtacgagacacggatcgacctgtctcagctgggaggcgacaaaaggccggcggccacgaaaaaggccggccaggcaaaaaagaaaaagtaagaattcgcccttcttcgttgaacaacggaaactcgacttgccttccgcacaatacatcatttcttcttagctttttttcttcttcttcgttcatacagtttttttttgtttatcagcttacattttcttgaaccgtagctttcgttttcttctttttaactttccattcggagtttttgtatcttgtttcatagtttgtcccaggattagaatgattaggcatcgaaccttcaagaatttgattgaataaaacatcttcattcttaagatatgaagataatcttcaaaaggcccctgggaatctgaaagaagagaagcaggcccatttatatgggaaagaacaatagtatttcttatataggcccatttaagttgaaaacaatcttcaaaagtcccacatcgcttagataagaaaacgaagctgagtttatatacagctagagtcgaagtagtgattgtgagaccgaggtctcggttttagagctagaaatagcaagttaaaataaggctagtccgttatcaacttgaaaaagtggcaccgagtcggtgcaacaaagcaccagtggtctagtggtagaatagtaccctgccacggtacagacccgggttcgattcccggctggtgcagcagatttggtatgatgtctgttttagagctagaaatagcaagttaaaataaggctagtccgttatcaacttgaaaaagtggcaccgagtcggtgcaacaaagcaccagtggtctagtggtagaatagtaccctgccacggtacagacccgggttcgattcccggctggtgcatggagctttatcctcgtatcgttttagagctagaaatagcaagttaaaataaggctagtccgttatcaacttgaaaaagtggcaccgagtcggtgctttttttctagagggcgaattcactggccgtcgttttacaacgtcgtgactgggaaaaccctggcgttacccaacttaatcgccttgcagcacatccccctttcgccagctggcgtaatagcgaagaggcccgcaccgatcgcccttcccaacagttgcgcagcctgaatggcgaatgctagagcagcttgagcttggatcagattgtcgtttcccgccttcagtttaaactatcagtgtttgacaggatatattggcgggtaaacctaagagaaaagagcgtttattagaataacggatatttaaaagggcgtgaaaaggtttatccgttcgtccatttgtatgtgcatgccaaccacagggttcccctcgggatcaaagtactttgatccaacccctccgctgctatagtgcagtcggcttctgacgttcagtgcagccgtcttctgaaaacgacatgtcgcacaagtcctaagttacgcgacaggctgccgccctgcccttttcctggcgttttcttgtcgcgtgttttagtcgcataaagtagaatacttgcgactagaaccggagacattacgccatgaacaagagcgccgccgctggcctgctgggctatgcccgcgtcagcaccgacgaccaggacttgaccaaccaacgggccgaactgcacgcggccggctgcaccaagctgttttccgagaagatcaccggcaccaggcgcgaccgcccggagctggccaggatgcttgaccacctacgccctggcgacgttgtgacagtgaccaggctagaccgcctggcccgcagcacccgcgacctactggacattgccgagcgcatccaggaggccggcgcgggcctgcgtagcctggcagagccgtgggccgacaccaccacgccggccggccgcatggtgttgaccgtgttcgccggcattgccgagttcgagcgttccctaatcatcgaccgcacccggagcgggcgcgaggccgccaaggcccgaggcgtgaagtttggcccccgccctaccctcaccccggcacagatcgcgcacgcccgcgagctgatcgaccaggaaggccgcaccgtgaaagaggcggctgcactgcttggcgtgcatcgctcgaccctgtaccgcgcacttgagcgcagcgaggaagtgacgcccaccgaggccaggcggcgcggtgccttccgtgaggacgcattgaccgaggccgacgccctggcggccgccgagaatgaacgccaagaggaacaagcatgaaaccgcaccaggacggccaggacgaaccgtttttcattaccgaagagatcgaggcggagatgatcgcggccgggtacgtgttcgagccgcccgcgcacgtctcaaccgtgcggctgcatgaaatcctggccggtttgtctgatgccaagctggcggcctggccggccagcttggccgctgaagaaaccgagcgccgccgtctaaaaaggtgatgtgtatttgagtaaaacagcttgcgtcatgcggtcgctgcgtatatgatgcgatgagtaaataaacaaatacgcaaggggaacgcatgaaggttatcgctgtacttaaccagaaaggcgggtcaggcaagacgaccatcgcaacccatctagcccgcgccctgcaactcgccggggccgatgttctgttagtcgattccgatccccagggcagtgcccgcgattgggcggccgtgcgggaagatcaaccgctaaccgttgtcggcatcgaccgcccgacgattgaccgcgacgtgaaggccatcggccggcgcgacttcgtagtgatcgacggagcgccccaggcggcggacttggctgtgtccgcgatcaaggcagccgacttcgtgctgattccggtgcagccaagcccttacgacatatgggccaccgccgacctggtggagctggttaagcagcgcattgaggtcacggatggaaggctacaagcggcctttgtcgtgtcgcgggcgatcaaaggcacgcgcatcggcggtgaggttgccgaggcgctggccgggtacgagctgcccattcttgagtcccgtatcacgcagcgcgtgagctacccaggcactgccgccgccggcacaaccgttcttgaatcagaacccgagggcgacgctgcccgcgaggtccaggcgctggccgctgaaattaaatcaaaactcatttgagttaatgaggtaaagagaaaatgagcaaaagcacaaacacgctaagtgccggccgtccgagcgcacgcagcagcaaggctgcaacgttggccagcctggcagacacgccagccatgaagcgggtcaactttcagttgccggcggaggatcacaccaagctgaagatgtacgcggtacgccaaggcaagaccattaccgagctgctatctgaatacatcgcgcagctaccagagtaaatgagcaaatgaataaatgagtagatgaattttagcggctaaaggaggcggcatggaaaatcaagaacaaccaggcaccgacgccgtggaatgccccatgtgtggaggaacgggcggttggccaggcgtaagcggctgggttgtctgccggccctgcaatggcactggaacccccaagcccgaggaatcggcgtgacggtcgcaaaccatccggcccggtacaaatcggcgcggcgctgggtgatgacctggtggagaagttgaaggccgcgcaggccgcccagcggcaacgcatcgaggcagaagcacgccccggtgaatcgtggcaagcggccgctgatcgaatccgcaaagaatcccggcaaccgccggcagccggtgcgccgtcgattaggaagccgcccaagggcgacgagcaaccagattttttcgttccgatgctctatgacgtgggcacccgcgatagtcgcagcatcatggacgtggccgttttccgtctgtcgaagcgtgaccgacgagctggcgaggtgatccgctacgagcttccagacgggcacgtagaggtttccgcagggccggccggcatggccagtgtgtgggattacgacctggtactgatggcggtttcccatctaaccgaatccatgaaccgataccgggaagggaagggagacaagcccggccgcgtgttccgtccacacgttgcggacgtactcaagttctgccggcgagccgatggcggaaagcagaaagacgacctggtagaaacctgcattcggttaaacaccacgcacgttgccatgcagcgtacgaagaaggccaagaacggccgcctggtgacggtatccgagggtgaagccttgattagccgctacaagatcgtaaagagcgaaaccgggcggccggagtacatcgagatcgagctagctgattggatgtaccgcgagatcacagaaggcaagaacccggacgtgctgacggttcaccccgattactttttgatcgatcccggcatcggccgttttctctaccgcctggcacgccgcgccgcaggcaaggcagaagccagatggttgttcaagacgatctacgaacgcagtggcagcgccggagagttcaagaagttctgtttcaccgtgcgcaagctgatcgggtcaaatgacctgccggagtacgatttgaaggaggaggcggggcaggctggcccgatcctagtcatgcgctaccgcaacctgatcgagggcgaagcatccgccggttcctaatgtacggagcagatgctagggcaaattgccctagcaggggaaaaaggtcgaaaagcactctttcctgtggatagcacgtacattgggaacccaaagccgtacattgggaaccggaacccgtacattgggaacccaaagccgtacattgggaaccggtcacacatgtaagtgactgatataaaagagaaaaaaggcgatttttccgcctaaaactctttaaaacttattaaaactcttaaaacccgcctggcctgtgcataactgtctggccagcgcacagccgaagagctgcaaaaagcgcctacccttcggtcgctgcgctccctacgccccgccgcttcgcgtcggcctatcgcggccgctggccgctcaaaaatggctggcctacggccaggcaatctaccagggcgcggacaagccgcgccgtcgccactcgaccgccggcgcccacatcaaggcaccctgcctcgcgcgtttcggtgatgacggtgaaaacctctgacacatgcagctcccggagacggtcacagcttgtctgtaagcggatgccgggagcagacaagcccgtcagggcgcgtcagcgggtgttggcgggtgtcggggcgcagccatgacccagtcacgtagcgatagcggagtgtatactggcttaactatgcggcatcagagcagattgtactgagagtgcaccatatgcggtgtgaaataccgcacagatgcgtaaggagaaaataccgcatcaggcgctcttccgcttcctcgctcactgactcgctgcgctcggtcgttcggctgcggcgagcggtatcagctcactcaaaggcggtaatacggttatccacagaatcaggggataacgcaggaaagaacatgtgagcaaaaggccagcaaaaggccaggaaccgtaaaaaggccgcgttgctggcgtttttccataggctccgcccccctgacgagcatcacaaaaatcgacgctcaagtcagaggtggcgaaacccgacaggactataaagataccaggcgtttccccctggaagctccctcgtgcgctctcctgttccgaccctgccgcttaccggatacctgtccgcctttctcccttcgggaagcgtggcgctttctcatagctcacgctgtaggtatctcagttcggtgtaggtcgttcgctccaagctgggctgtgtgcacgaaccccccgttcagcccgaccgctgcgccttatccggtaactatcgtcttgagtccaacccggtaagacacgacttatcgccactggcagcagccactggtaacaggattagcagagcgaggtatgtaggcggtgctacagagttcttgaagtggtggcctaactacggctacactagaaggacagtatttggtatctgcgctctgctgaagccagttaccttcggaaaaagagttggtagctcttgatccggcaaacaaaccaccgctggtagcggtggtttttttgtttgcaagcagcagattacgcgcagaaaaaaaggatctcaagaagatcctttgatcttttctacggggtctgacgctcagtggaacgaaaactcacgttaagggattttggtcatgcattctaggtactaaaacaattcatccagtaaaatataatattttattttctcccaatcaggcttgatccccagtaagtcaaaaaatagctcgacatactgttcttccccgatatcctccctgatcgaccggacgcagaaggcaatgtcataccacttgtccgccctgccgcttctcccaagatcaataaagccacttactttgccatctttcacaaagatgttgctgtctcccaggtcgccgtgggaaaagacaagttcctcttcgggcttttccgtctttaaaaaatcatacagctcgcgcggatctttaaatggagtgtcttcttcccagttttcgcaatccacatcggccagatcgttattcagtaagtaatccaattcggctaagcggctgtctaagctattcgtatagggacaatccgatatgtcgatggagtgaaagagcctgatgcactccgcatacagctcgataatcttttcagggctttgttcatcttcatactcttccgagcaaaggacgccatcggcctcactcatgagcagattgctccagccatcatgccgttcaaagtgcaggacctttggaacaggcagctttccttccagccatagcatcatgtccttttcccgttccacatcataggtggtccctttataccggctgtccgtcatttttaaatataggttttcattttctcccaccagcttatataccttagcaggagacattccttccgtatcttttacgcagcggtatttttcgatcagttttttcaattccggtgatattctcattttagccatttattatttccttcctcttttctacagtatttaaagataccccaagaagctaattataacaagacgaactccaattcactgttccttgcattctaaaaccttaaataccagaaaacagctttttcaaagttgttttcaaagttggcgtataacatagtatcgacggagccgattttgaaaccgcggtgatcacaggcagcaacgctctgtcatcgttacaatcaacatgctaccctccgcgagatcatccgtgtttcaaacccggcagcttagttgccgttcttccgaatagcatcggtaacatgagcaaagtctgccgccttacaacggctctcccgctgacgccgtcccggactgatgggctgcctgtatcgagtggtgattttgtgccgagctgccggtcggggagctgttggctggctggtggcaggatatattgtggtgtaaacaaattgacgcttagacaacttaataacacattgcggacgtttttaatgtactgaattaacgccgaattaattcgggggatctggattttagtactggattttggttttaggaattagaaattttattgatagaagtattttacaaatacaaatacatactaagggtttcttatatgctcaacacatgagcgaaaccctataggaaccctaattcccttatctgggaactactcacacattattatggagaaactcgagcttgtcgatcgacagatccggtcggcatctactctatttctttgccctcggacgagtgctggggcgtcggtttccactatcggcgagtacttctacacagccatcggtccagacggccgcgcttctgcgggcgatttgtgtacgcccgacagtcccggctccggatcggacgattgcgtcgcatcgaccctgcgcccaagctgcatcatcgaaattgccgtcaaccaagctctgatagagttggtcaagaccaatgcggagcatatacgcccggagtcgtggcgatcctgcaagctccggatgcctccgctcgaagtagcgcgtctgctgctccatacaagccaaccacggcctccagaagaagatgttggcgacctcgtattgggaatccccgaacatcgcctcgctccagtcaatgaccgctgttatgcggccattgtccgtcaggacattgttggagccgaaatccgcgtgcacgaggtgccggacttcggggcagtcctcggcccaaagcatcagctcatcgagagcctgcgcgacggacgcactgacggtgtcgtccatcacagtttgccagtgatacacatggggatcagcaatcgcgcatatgaaatcacgccatgtagtgtattgaccgattccttgcggtccgaatgggccgaacccgctcgtctggctaagatcggccgcagcgatcgcatccatagcctccgcgaccggttgtagaacagcgggcagttcggtttcaggcaggtcttgcaacgtgacaccctgtgcacggcgggagatgcaataggtcaggctctcgctaaactccccaatgtcaagcacttccggaatcgggagcgcggccgatgcaaagtgccgataaacataacgatctttgtagaaaccatcggcgcagctatttacccgcaggacatatccacgccctcctacatcgaagctgaaagcacgagattcttcgccctccgagagctgcatcaggtcggagacgctgtcgaacttttcgatcagaaacttctcgacagacgtcgcggtgagttcaggctttttcatatctcattgccccccgggatctgcgaaagctcgagagagatagatttgtagagagagactggtgatttcagcgtgtcctctccaaatgaaatgaacttccttatatagaggaaggtcttgcgaaggatagtgggattgtgcgtcatcccttacgtcagtggagatatcacatcaatccacttgctttgaagacgtggttggaacgtcttctttttccacgatgctcctcgtgggtgggggtccatctttgggaccactgtcggcagaggcatcttgaacgatagcctttcctttatcgcaatgatggcatttgtaggtgccaccttccttttctactgtccttttgatgaagtgacagatagctgggcaatggaatccgaggaggtttcccgatattaccctttgttgaaaagtctcaatagccctttggtcttctgagactgtatctttgatattcttggagtagacgagagtgtcgtgctccaccatgttatcacatcaatccacttgctttgaagacgtggttggaacgtcttctttttccacgatgctcctcgtgggtgggggtccatctttgggaccactgtcggcagaggcatcttgaacgatagcctttcctttatcgcaatgatggcatttgtaggtgccaccttccttttctactgtccttttgatgaagtgacagatagctgggcaatggaatccgaggaggtttcccgatattaccctttgttgaaaagtctcaatagccctttggtcttctgagactgtatctttgatattcttggagtagacgagagtgtcgtgctccaccatgttggcaagctgctctagccaatacgcaaaccgcctctccccgcgcgttggccgattcattaatgcagctggcacgacaggtttcccgactggaaagcgggcagtgagcgcaacgcaattaatgtgagttagctcactcattaggcaccccaggctttacactttatgcttccggctcgtatgttgtgtggaattgtgagcggataacaatttcacacaggaaacagctatgaccatgattacgcc

SEQ ID NO: 37 - DNA, 16300 bp, synthetic construct
  misc_feature 1..16300: note = nucleotides coding D120
  source 1..16300: mol_type = other DNA
aagcttgataatttatttgaaaattcataagaaaagcaaacgttacatgaattgatgaaacaatacaaagacagataaagccacgcacatttaggatattggccgagattactgaatattgagtaagatcacggaatttctgacaggagcatgtcttcaattcagcccaaatggcagttgaaatactcaaaccgccccatatgcaggagcggatcattcattgtttgtttggttgcctttgccaacatgggagtccaagattctgcagtcaaatctcggtgacgggcaggaccggacggggcggtaccggcaggctgaagtccagctgccagaaacccacgtcatgccagttcccgtgcttgaagccggccgcccgcagcatgccgcggggggcatatccgagcgcctcgtgcatgcgcacgctcgggtcgttgggcagcccgatgacagcgaccacgctcttgaagccctgtgcctccagggacttcagcaggtgggtgtagagcgtggagcccagtcccgtccgctggtggcggggggagacgtacacggtcgactcggccgtccagtcgtaggcgttgcgtgccttccaggggcccgcgtaggcgatgccggcgacctcgccgtccacctcggcgacgagccagggatagcgctcccgcagacggacgaggtcgtccgtccactcctgcggttcctgcggctcggtacggaagttgaccgtgcttgtctcgatgtagtggttgacgatggtgcagaccgccggcatgtccgcctcggtggcacggcggatgtcggccgggcgtcgttctgggctcatcgattcgatttggtgtatcgagattggttatgaaattcagatgctagtgtaatgtattggtaatttgggaagatataataggaagcaaggctatttatccatttctgaaaaggcgaaatggcgtcaccgcgagcgtcacgcgcattccgttcttgctgtaaagcgttgtttggtacacttttgactagcgaggcttggcgtgtcagcgtatctattcaaaagtcgttaatggctgcggatcaagaaaaagttggaatagaaacagaatacccgcgaaattcaggcccggttgccatgtcctacacgccgaaataaacgaccaaattagtagaaaaataaaaactgactcggatacttacgtcacgtcttgcgcactgatttgaaaaatctcagccatggctgcaggtcgacgagtcagtaataaacggcgtcaaagtggttgcagccggcacacacgagtcgtgtttatcaactcaaagcacaaatacttttcctcaacctaaaaataaggcaattagccaaaaacaactttgcgtgtaaacaacgctcaatacacgtgtcattttattattagctattgcttcaccgccttagctttctcgtgacctagtcgtcctcgtcttttcttcttcttcttctataaaacaatacccaaagagctcttcttcttcacaattcagatttcaatttctcaaaatcttaaaaactttctctcaattctctctaccgtgatcaaggtaaatttctgtgttccttattctctcaaaatcttcgattttgttttcgttcgatcccaatttcgtatatgttctttggtttagattctgttaatcttagatcgaagacgattttctgggtttgatcgttagatatcatcttaattctcgattagggtttcatagatatcatccgatttgttcaaataatttgagttttgtcgaataattactcttcgatttgtgatttctatctagatctggtgttagtttctagtttgtgcgatcgaatttgtcgattaatctgagtttttctgattaacagccatggactataaggaccacgacggagactacaaggatcatgatattgattacaaagacgatgacgataagatggccccaaagaagaagcggaaggtcggtatccacggagtcccagcagccgacaagaagtacagcatcggcctggacatcggcaccaactctgtgggctgggccgtgatcaccgacgagtacaaggtgcccagcaagaaattcaaggtgctgggcaacaccgaccggcacagcatcaagaagaacctgatcggagccctgctgttcgacagcggcgaaacagccgaggccacccggctgaagagaaccgccagaagaagatacaccagacggaagaaccggatctgctatctgcaagagatcttcagcaacgagatggccaaggtggacgacagcttcttccacagactggaagagtccttcctggtggaagaggataagaagcacgagcggcaccccatcttcggcaacatcgtggacgaggtggcctaccacgagaagtaccccaccatctaccacctgagaaagaaactggtggacagcaccgacaaggccgacctgcggctgatctatctggccctggcccacatgatcaagttccggggccacttcctgatcgagggcgacctgaaccccgacaacagcgacgtggacaagctgttcatccagctggtgcagacctacaaccagctgttcgaggaaaaccccatcaacgccagcggcgtggacgccaaggccatcctgtctgccagactgagcaagagcagacggctggaaaatctgatcgcccagctgcccggcgagaagaagaatggcctgttcggaaacctgattgccctgagcctgggcctgacccccaacttcaagagcaacttcgacctggccgaggatgccaaactgcagctgagcaaggacacctacgacgacgacctggacaacctgctggcccagatcggcgaccagtacgccgacctgtttctggccgccaagaacctgtccgacgccatcctgctgagcgacatcctgagagtgaacaccgagatcaccaaggcccccctgagcgcctctatgatcaagagatacgacgagcaccaccaggacctgaccctgctgaaagctctcgtgcggcagcagctgcctgagaagtacaaagagattttcttcgaccagagcaagaacggctacgccggctacattgacggcggagccagccaggaagagttctacaagttcatcaagcccatcctggaaaagatggacggcaccgaggaactgctcgtgaagctgaacagagaggacctgctgcggaagcagcggaccttcgacaacggcagcatcccccaccagatccacctgggagagctgcacgccattctgcggcggcaggaagatttttacccattcctgaaggacaaccgggaaaagatcgagaagatcctgaccttccgcatcccctactacgtgggccctctggccaggggaaacagcagattcgcctggatgaccagaaagagcgaggaaaccatcaccccctggaacttcgaggaagtggtggacaagggcgcttccgcccagagcttcatcgagcggatgaccaacttcgataagaacctgcccaacgagaaggtgctgcccaagcacagcctgctgtacgagtacttcaccgtgtataacgagctgaccaaagtgaaatacgtgaccgagggaatgagaaagcccgccttcctgagcggcgagcagaaaaaggccatcgtggacctgctgttcaagaccaaccggaaagtgaccgtgaagcagctgaaagaggactacttcaagaaaatcgagtgcttcgactccgtggaaatctccggcgtggaagatcggttcaacgcctccctgggcacataccacgatctgctgaaaattatcaaggacaaggacttcctggacaatgaggaaaacgaggacattctggaagatatcgtgctgaccctgacactgtttgaggacagagagatgatcgaggaacggctgaaaacctatgcccacctgttcgacgacaaagtgatgaagcagctgaagcggcggagatacaccggctggggcaggctgagccggaagctgatcaacggcatccgggacaagcagtccggcaagacaatcctggatttcctgaagtccgacggcttcgccaacagaaacttcatgcagctgatccacgacgacagcctgacctttaaagaggacatccagaaagcccaggtgtccggccagggcgatagcctgcacgagcacattgccaatctggccggcagccccgccattaagaagggcatcctgcagacagtgaaggtggtggacgagctcgtgaaagtgatgggccggcacaagcccgagaacatcgtgatcgaaatggccagagagaaccagaccacccagaagggacagaagaacagccgcgagagaatgaagcggatcgaagagggcatcaaagagctgggcagccagatcctgaaagaacaccccgtggaaaacacccagctgcagaacgagaagctgtacctgtactacctgcagaatgggcgggatatgtacgtggaccaggaactggacatcaaccggctgtccgactacgatgtggaccatatcgtgcctcagagctttctgaaggacgactccatcgacaacaaggtgctgaccagaagcgacaagaaccggggcaagagcgacaacgtgccctccgaagaggtcgtgaagaagatgaagaactactggcggcagctgctgaacgccaagctgattacccagagaaagttcgacaatctgaccaaggccgagagaggcggcctgagcgaactggataaggccggcttcatcaagagacagctggtggaaacccggcagatcacaaagcacgtggcacagatcctggactcccggatgaacactaagtacgacgagaatgacaagctgatccgggaagtgaaagtgatcaccctgaagtccaagctggtgtccgatttccggaaggatttccagttttacaaagtgcgcgagatcaacaactaccaccacgcccacgacgcctacctgaacgccgtcgtgggaaccgccctgatcaaaaagtaccctaagctggaaagcgagttcgtgtacggcgactacaaggtgtacgacgtgcggaagatgatcgccaagagcgagcaggaaatcggcaaggctaccgccaagtacttcttctacagcaacatcatgaactttttcaagaccgagattaccctggccaacggcgagatccggaagcggcctctgatcgagacaaacggcgaaaccggggagatcgtgtgggataagggccgggattttgccaccgtgcggaaagtgctgagcatgccccaagtgaatatcgtgaaaaagaccgaggtgcagacaggcggcttcagcaaagagtctatcctgcccaagaggaacagcgataagctgatcgccagaaagaaggactgggaccctaagaagtacggcggcttcgacagccccaccgtggcctattctgtgctggtggtggccaaagtggaaaagggcaagtccaagaaactgaagagtgtgaaagagctgctggggatcaccatcatggaaagaagcagcttcgagaagaatcccatcgactttctggaagccaagggctacaaagaagtgaaaaaggacctgatcatcaagctgcctaagtactccctgttcgagctggaaaacggccggaagagaatgctggcctctgccggcgaactgcagaagggaaacgaactggccctgccctccaaatatgtgaacttcctgtacctggccagccactatgagaagctgaagggctcccccgaggataatgagcagaaacagctgtttgtggaacagcacaagcactacctggacgagatcatcgagcagatcagcgagttctccaagagagtgatcctggccgacgctaatctggacaaagtgctgtccgcctacaacaagcaccgggataagcccatcagagagcaggccgagaatatcatccacctgtttaccctgaccaatctgggagcccctgccgccttcaagtactttgacaccaccatcgaccggaagaggtacaccagcaccaaagaggtgctggacgccaccctgatccaccagagcatcaccggcctgtacgagacacggatcgacctgtctcagctgggaggcgacaaaaggccggcggccacgaaaaaggccggccaggcaaaaaagaaaaagtaagaattcgcccttcttcgttgaacaacggaaactcgacttgccttccgcacaatacatcatttcttcttagctttttttcttcttcttcgttcatacagtttttttttgtttatcagcttacattttcttgaaccgtagctttcgttttcttctttttaactttccattcggagtttttgtatcttgtttcatagtttgtcccaggattagaatgattaggcatcgaaccttcaagaatttgattgaataaaacatcttcattcttaagatatgaagataatcttcaaaaggcccctgggaatctgaaagaagagaagcaggcccatttatatgggaaagaacaatagtatttcttatataggcccatttaagttgaaaacaatcttcaaaagtcccacatcgcttagataagaaaacgaagctgagtttatatacagctagagtcgaagtagtgattgtgagaccgaggtctcggttttagagctagaaatagcaagttaaaataaggctagtccgttatcaacttgaaaaagtggcaccgagtcggtgcaacaaagcaccagtggtctagtggtagaatagtaccctgccacggtacagacccgggttcgattcccggctggtgcatgagcagaaagaagaagagagttttagagctagaaatagcaagttaaaataaggctagtccgttatcaacttgaaaaagtggcaccgagtcggtgcaacaaagcaccagtggtctagtggtagaatagtaccctgccacggtacagacccgggttcgattcccggctggtgcacgcttcagcatccttgtcgtgttttagagctagaaatagcaagttaaaataaggctagtccgttatcaacttgaaaaagtggcaccgagtcggtgcaacaaagcaccagtggtctagtggtagaatagtaccctgccacggtacagacccgggttcgattcccggctggtgcagcagatttggtatgatgtctgttttagagctagaaatagcaagttaaaataaggctagtccgttatcaacttgaaaaagtggcaccgagtcggtgcaacaaagcaccagtggtctagtggtagaatagtaccctgccacggtacagacccgggttcgattcccggctggtgcatggagctttatcctcgtatcgttttagagctagaaatagcaagttaaaataaggctagtccgttatcaacttgaaaaagtggcaccgagtcggtgctttttttctagagggcgaattcactggccgtcgttttacaacgtcgtgactgggaaaaccctggcgttacccaacttaatcgccttgcagcacatccccctttcgccagctggcgtaatagcgaagaggcccgcaccgatcgcccttcccaacagttgcgcagcctgaatggcgaatgctagagcagcttgagcttggatcagattgtcgtttcccgccttcagtttaaactatcagtgtttgacaggatatattggcgggtaaacctaagagaaaagagcgtttattagaataacggatatttaaaagggcgtgaaaaggtttatccgttcgtccatttgtatgtgcatgccaaccacagggttcccctcgggatcaaagtactttgatccaacccctccgctgctatagtgcagtcggcttctgacgttcagtgcagccgtcttctgaaaacgacatgtcgcacaagtcctaagttacgcgacaggctgccgccctgcccttttcctggcgttttcttgtcgcgtgttttagtcgcataaagtagaatacttgcgactagaaccggagacattacgccatgaacaagagcgccgccgctggcctgctgggctatgcccgcgtcagcaccgacgaccaggacttgaccaaccaacgggccgaactgcacgcggccggctgcaccaagctgttttccgagaagatcaccggcaccaggcgcgaccgcccggagctggccaggatgcttgaccacctacgccctggcgacgttgtgacagtgaccaggctagaccgcctggcccgcagcacccgcgacctactggacattgccgagcgcatccaggaggccggcgcgggcctgcgtagcctggcagagccgtgggccgacaccaccacgccggccggccgcatggtgttgaccgtgttcgccggcattgccgagttcgagcgttccctaatcatcgaccgcacccggagcgggcgcgaggccgccaaggcccgaggcgtgaagtttggcccccgccctaccctcaccccggcacagatcgcgcacgcccgcgagctgatcgaccaggaaggccgcaccgtgaaagaggcggctgcactgcttggcgtgcatcgctcgaccctgtaccgcgcacttgagcgcagcgaggaagtgacgcccaccgaggccaggcggcgcggtgccttccgtgaggacgcattgaccgaggccgacgccctggcggccgccgagaatgaacgccaagaggaacaagcatgaaaccgcaccaggacggccaggacgaaccgtttttcattaccgaagagatcgaggcggagatgatcgcggccgggtacgtgttcgagccgcccgcgcacgtctcaaccgtgcggctgcatgaaatcctggccggtttgtctgatgccaagctggcggcctggccggccagcttggccgctgaagaaaccgagcgccgccgtctaaaaaggtgatgtgtatttgagtaaaacagcttgcgtcatgcggtcgctgcgtatatgatgcgatgagtaaataaacaaatacgcaaggggaacgcatgaaggttatcgctgtacttaaccagaaaggcgggtcaggcaagacgaccatcgcaacccatctagcccgcgccctgcaactcgccggggccgatgttctgttagtcgattccgatccccagggcagtgcccgcgattgggcggccgtgcgggaagatcaaccgctaaccgttgtcggcatcgaccgcccgacgattgaccgcgacgtgaaggccatcggccggcgcgacttcgtagtgatcgacggagcgccccaggcggcggacttggctgtgtccgcgatcaaggcagccgacttcgtgctgattccggtgcagccaagcccttacgacatatgggccaccgccgacctggtggagctggttaagcagcgcattgaggtcacggatggaaggctacaagcggcctttgtcgtgtcgcgggcgatcaaaggcacgcgcatcggcggtgaggttgccgaggcgctggccgggtacgagctgcccattcttgagtcccgtatcacgcagcgcgtgagctacccaggcactgccgccgccggcacaaccgttcttgaatcagaacccgagggcgacgctgcccgcgaggtccaggcgctggccgctgaaattaaatcaaaactcatttgagttaatgaggtaaagagaaaatgagcaaaagcacaaacacgctaagtgccggccgtccgagcgcacgcagcagcaaggctgcaacgttggccagcctggcagacacgccagccatgaagcgggtcaactttcagttgccggcggaggatcacaccaagctgaagatgtacgcggtacgccaaggcaagaccattaccgagctgctatctgaatacatcgcgcagctaccagagtaaatgagcaaatgaataaatgagtagatgaattttagcggctaaaggaggcggcatggaaaatcaagaacaaccaggcaccgacgccgtggaatgccccatgtgtggaggaacgggcggttggccaggcgtaagcggctgggttgtctgccggccctgcaatggcactggaacccccaagcccgaggaatcggcgtgacggtcgcaaaccatccggcccggtacaaatcggcgcggcgctgggtgatgacctggtggagaagttgaaggccgcgcaggccgcccagcggcaacgcatcgaggcagaagcacgccccggtgaatcgtggcaagcggccgctgatcgaatccgcaaagaatcccggcaaccgccggcagccggtgcgccgtcgattaggaagccgcccaagggcgacgagcaaccagattttttcgttccgatgctctatgacgtgggcacccgcgatagtcgcagcatcatggacgtggccgttttccgtctgtcgaagcgtgaccgacgagctggcgaggtgatccgctacgagcttccagacgggcacgtagaggtttccgcagggccggccggcatggccagtgtgtgggattacgacctggtactgatggcggtttcccatctaaccgaatccatgaaccgataccgggaagggaagggagacaagcccggccgcgtgttccgtccacacgttgcggacgtactcaagttctgccggcgagccgatggcggaaagcagaaagacgacctggtagaaacctgcattcggttaaacaccacgcacgttgccatgcagcgtacgaagaaggccaagaacggccgcctggtgacggtatccgagggtgaagccttgattagccgctacaagatcgtaaagagcgaaaccgggcggccggagtacatcgagatcgagctagctgattggatgtaccgcgagatcacagaaggcaagaacccggacgtgctgacggttcaccccgattactttttgatcgatcccggcatcggccgttttctctaccgcctggcacgccgcgccgcaggcaaggcagaagccagatggttgttcaagacgatctacgaacgcagtggcagcgccggagagttcaagaagttctgtttcaccgtgcgcaagctgatcgggtcaaatgacctgccggagtacgatttgaaggaggaggcggggcaggctggcccgatcctagtcatgcgctaccgcaacctgatcgagggcgaagcatccgccggttcctaatgtacggagcagatgctagggcaaattgccctagcaggggaaaaaggtcgaaaagcactctttcctgtggatagcacgtacattgggaacccaaagccgtacattgggaaccggaacccgtacattgggaacccaaagccgtacattgggaaccggtcacacatgtaagtgactgatataaaagagaaaaaaggcgatttttccgcctaaaactctttaaaacttattaaaactcttaaaacccgcctggcctgtgcataactgtctggccagcgcacagccgaagagctgcaaaaagcgcctacccttcggtcgctgcgctccctacgccccgccgcttcgcgtcggcctatcgcggccgctggccgctcaaaaatggctggcctacggccaggcaatctaccagggcgcggacaagccgcgccgtcgccactcgaccgccggcgcccacatcaaggcaccctgcctcgcgcgtttcggtgatgacggtgaaaacctctgacacatgcagctcccggagacggtcacagcttgtctgtaagcggatgccgggagcagacaagcccgtcagggcgcgtcagcgggtgttggcgggtgtcggggcgcagccatgacccagtcacgtagcgatagcggagtgtatactggcttaactatgcggcatcagagcagattgtactgagagtgcaccatatgcggtgtgaaataccgcacagatgcgtaaggagaaaataccgcatcaggcgctcttccgcttcctcgctcactgactcgctgcgctcggtcgttcggctgcggcgagcggtatcagctcactcaaaggcggtaatacggttatccacagaatcaggggataacgcaggaaagaacatgtgagcaaaaggccagcaaaaggccaggaaccgtaaaaaggccgcgttgctggcgtttttccataggctccgcccccctgacgagcatcacaaaaatcgacgctcaagtcagaggtggcgaaacccgacaggactataaagataccaggcgtttccccctggaagctccctcgtgcgctctcctgttccgaccctgccgcttaccggatacctgtccgcctttctcccttcgggaagcgtggcgctttctcatagctcacgctgtaggtatctcagttcggtgtaggtcgttcgctccaagctgggctgtgtgcacgaaccccccgttcagcccgaccgctgcgccttatccggtaactatcgtcttgagtccaacccggtaagacacgacttatcgccactggcagcagccactggtaacaggattagcagagcgaggtatgtaggcggtgctacagagttcttgaagtggtggcctaactacggctacactagaaggacagtatttggtatctgcgctctgctgaagccagttaccttcggaaaaagagttggtagctcttgatccggcaaacaaaccaccgctggtagcggtggtttttttgtttgcaagcagcagattacgcgcagaaaaaaaggatctcaagaagatcctttgatcttttctacggggtctgacgctcagtggaacgaaaactcacgttaagggattttggtcatgcattctaggtactaaaacaattcatccagtaaaatataatattttattttctcccaatcaggcttgatccccagtaagtcaaaaaatagctcgacatactgttcttccccgatatcctccctgatcgaccggacgcagaaggcaatgtcataccacttgtccgccctgccgcttctcccaagatcaataaagccacttactttgccatctttcacaaagatgttgctgtctcccaggtcgccgtgggaaaagacaagttcctcttcgggcttttccgtctttaaaaaatcatacagctcgcgcggatctttaaatggagtgtcttcttcccagttttcgcaatccacatcggccagatcgttattcagtaagtaatccaattcggctaagcggctgtctaagctattcgtatagggacaatccgatatgtcgatggagtgaaagagcctgatgcactccgcatacagctcgataatcttttcagggctttgttcatcttcatactcttccgagcaaaggacgccatcggcctcactcatgagcagattgctccagccatcatgccgttcaaagtgcaggacctttggaacaggcagctttccttccagccatagcatcatgtccttttcccgttccacatcataggtggtccctttataccggctgtccgtcatttttaaatataggttttcattttctcccaccagcttatataccttagcaggagacattccttccgtatcttttacgcagcggtatttttcgatcagttttttcaattccggtgatattctcattttagccatttattatttccttcctcttttctacagtatttaaagataccccaagaagctaattataacaagacgaactccaattcactgttccttgcattctaaaaccttaaataccagaaaacagctttttcaaagttgttttcaaagttggcgtataacatagtatcgacggagccgattttgaaaccgcggtgatcacaggcagcaacgctctgtcatcgttacaatcaacatgctaccctccgcgagatcatccgtgtttcaaacccggcagcttagttgccgttcttccgaatagcatcggtaacatgagcaaagtctgccgccttacaacggctctcccgctgacgccgtcccggactgatgggctgcctgtatcgagtggtgattttgtgccgagctgccggtcggggagctgttggctggctggtggcaggatatattgtggtgtaaacaaattgacgcttagacaacttaataacacattgcggacgtttttaatgtactgaattaacgccgaattaattcgggggatctggattttagtactggattttggttttaggaattagaaattttattgatagaagtattttacaaatacaaatacatactaagggtttcttatatgctcaacacatgagcgaaaccctataggaaccctaattcccttatctgggaactactcacacattattatggagaaactcgagcttgtcgatcgacagatccggtcggcatctactctatttctttgccctcggacgagtgctggggcgtcggtttccactatcggcgagtacttctacacagccatcggtccagacggccgcgcttctgcgggcgatttgtgtacgcccgacagtcccggctccggatcggacgattgcgtcgcatcgaccctgcgcccaagctgcatcatcgaaattgccgtcaaccaagctctgatagagttggtcaagaccaatgcggagcatatacgcccggagtcgtggcgatcctgcaagctccggatgcctccgctcgaagtagcgcgtctgctgctccatacaagccaaccacggcctccagaagaagatgttggcgacctcgtattgggaatccccgaacatcgcctcgctccagtcaatgaccgctgttatgcggccattgtccgtcaggacattgttggagccgaaatccgcgtgcacgaggtgccggacttcggggcagtcctcggcccaaagcatcagctcatcgagagcctgcgcgacggacgcactgacggtgtcgtccatcacagtttgccagtgatacacatggggatcagcaatcgcgcatatgaaatcacgccatgtagtgtattgaccgattccttgcggtccgaatgggccgaacccgctcgtctggctaagatcggccgcagcgatcgcatccatagcctccgcgaccggttgtagaacagcgggcagttcggtttcaggcaggtcttgcaacgtgacaccctgtgcacggcgggagatgcaataggtcaggctctcgctaaactccccaatgtcaagcacttccggaatcgggagcgcggccgatgcaaagtgccgataaacataacgatctttgtagaaaccatcggcgcagctatttacccgcaggacatatccacgccctcctacatcgaagctgaaagcacgagattcttcgccctccgagagctgcatcaggtcggagacgctgtcgaacttttcgatcagaaacttctcgacagacgtcgcggtgagttcaggctttttcatatctcattgccccccgggatctgcgaaagctcgagagagatagatttgtagagagagactggtgatttcagcgtgtcctctccaaatgaaatgaacttccttatatagaggaaggtcttgcgaaggatagtgggattgtgcgtcatcccttacgtcagtggagatatcacatcaatccacttgctttgaagacgtggttggaacgtcttctttttccacgatgctcctcgtgggtgggggtccatctttgggaccactgtcggcagaggcatcttgaacgatagcctttcctttatcgcaatgatggcatttgtaggtgccaccttccttttctactgtccttttgatgaagtgacagatagctgggcaatggaatccgaggaggtttcccgatattaccctttgttgaaaagtctcaatagccctttggtcttctgagactgtatctttgatattcttggagtagacgagagtgtcgtgctccaccatgttatcacatcaatccacttgctttgaagacgtggttggaacgtcttctttttccacgatgctcctcgtgggtgggggtccatctttgggaccactgtcggcagaggcatcttgaacgatagcctttcctttatcgcaatgatggcatttgtaggtgccaccttccttttctactgtccttttgatgaagtgacagatagctgggcaatggaatccgaggaggtttcccgatattaccctttgttgaaaagtctcaatagccctttggtcttctgagactgtatctttgatattcttggagtagacgagagtgtcgtgctccaccatgttggcaagctgctctagccaatacgcaaaccgcctctccccgcgcgttggccgattcattaatgcagctggcacgacaggtttcccgactggaaagcgggcagtgagcgcaacgcaattaatgtgagttagctcactcattaggcaccccaggctttacactttatgcttccggctcgtatgttgtgtggaattgtgagcggataacaatttcacacaggaaacagctatgaccatgattacgcc

SEQ ID NO: 38 - DNA, 16477 bp, synthetic construct
  misc_feature 1..16477: note = nucleotides coding D121
  source 1..16477: mol_type = other DNA
aagcttgataatttatttgaaaattcataagaaaagcaaacgttacatgaattgatgaaacaatacaaagacagataaagccacgcacatttaggatattggccgagattactgaatattgagtaagatcacggaatttctgacaggagcatgtcttcaattcagcccaaatggcagttgaaatactcaaaccgccccatatgcaggagcggatcattcattgtttgtttggttgcctttgccaacatgggagtccaagattctgcagtcaaatctcggtgacgggcaggaccggacggggcggtaccggcaggctgaagtccagctgccagaaacccacgtcatgccagttcccgtgcttgaagccggccgcccgcagcatgccgcggggggcatatccgagcgcctcgtgcatgcgcacgctcgggtcgttgggcagcccgatgacagcgaccacgctcttgaagccctgtgcctccagggacttcagcaggtgggtgtagagcgtggagcccagtcccgtccgctggtggcggggggagacgtacacggtcgactcggccgtccagtcgtaggcgttgcgtgccttccaggggcccgcgtaggcgatgccggcgacctcgccgtccacctcggcgacgagccagggatagcgctcccgcagacggacgaggtcgtccgtccactcctgcggttcctgcggctcggtacggaagttgaccgtgcttgtctcgatgtagtggttgacgatggtgcagaccgccggcatgtccgcctcggtggcacggcggatgtcggccgggcgtcgttctgggctcatcgattcgatttggtgtatcgagattggttatgaaattcagatgctagtgtaatgtattggtaatttgggaagatataataggaagcaaggctatttatccatttctgaaaaggcgaaatggcgtcaccgcgagcgtcacgcgcattccgttcttgctgtaaagcgttgtttggtacacttttgactagcgaggcttggcgtgtcagcgtatctattcaaaagtcgttaatggctgcggatcaagaaaaagttggaatagaaacagaatacccgcgaaattcaggcccggttgccatgtcctacacgccgaaataaacgaccaaattagtagaaaaataaaaactgactcggatacttacgtcacgtcttgcgcactgatttgaaaaatctcagccatggctgcaggtcgacgagtcagtaataaacggcgtcaaagtggttgcagccggcacacacgagtcgtgtttatcaactcaaagcacaaatacttttcctcaacctaaaaataaggcaattagccaaaaacaactttgcgtgtaaacaacgctcaatacacgtgtcattttattattagctattgcttcaccgccttagctttctcgtgacctagtcgtcctcgtcttttcttcttcttcttctataaaacaatacccaaagagctcttcttcttcacaattcagatttcaatttctcaaaatcttaaaaactttctctcaattctctctaccgtgatcaaggtaaatttctgtgttccttattctctcaaaatcttcgattttgttttcgttcgatcccaatttcgtatatgttctttggtttagattctgttaatcttagatcgaagacgattttctgggtttgatcgttagatatcatcttaattctcgattagggtttcatagatatcatccgatttgttcaaataatttgagttttgtcgaataattactcttcgatttgtgatttctatctagatctggtgttagtttctagtttgtgcgatcgaatttgtcgattaatctgagtttttctgattaacagccatggactataaggaccacgacggagactacaaggatcatgatattgattacaaagacgatgacgataagatggccccaaagaagaagcggaaggtcggtatccacggagtcccagcagccgacaagaagtacagcatcggcctggacatcggcaccaactctgtgggctgggccgtgatcaccgacgagtacaaggtgcccagcaagaaattcaaggtgctgggcaacaccgaccggcacagcatcaagaagaacctgatcggagccctgctgttcgacagcggcgaaacagccgaggccacccggctgaagagaaccgccagaagaagatacaccagacggaagaaccggatctgctatctgcaagagatcttcagcaacgagatggccaaggtggacgacagcttcttccacagactggaagagtccttcctggtggaagaggataagaagcacgagcggcaccccatcttcggcaacatcgtggacgaggtggcctaccacgagaagtaccccaccatctaccacctgagaaagaaactggtggacagcaccgacaaggccgacctgcggctgatctatctggccctggcccacatgatcaagttccggggccacttcctgatcgagggcgacctgaaccccgacaacagcgacgtggacaagctgttcatccagctggtgcagacctacaaccagctgttcgaggaaaaccccatcaacgccagcggcgtggacgccaaggccatcctgtctgccagactgagcaagagcagacggctggaaaatctgatcgcccagctgcccggcgagaagaagaatggcctgttcggaaacctgattgccctgagcctgggcctgacccccaacttcaagagcaacttcgacctggccgaggatgccaaactgcagctgagcaaggacacctacgacgacgacctggacaacctgctggcccagatcggcgaccagtacgccgacctgtttctggccgccaagaacctgtccgacgccatcctgctgagcgacatcctgagagtgaacaccgagatcaccaaggcccccctgagcgcctctatgatcaagagatacgacgagcaccaccaggacctgaccctgctgaaagctctcgtgcggcagcagctgcctgagaagtacaaagagattttcttcgaccagagcaagaacggctacgccggctacattgacggcggagccagccaggaagagttctacaagttcatcaagcccatcctggaaaagatggacggcaccgaggaactgctcgtgaagctgaacagagaggacctgctgcggaagcagcggaccttcgacaacggcagcatcccccaccagatccacctgggagagctgcacgccattctgcggcggcaggaagatttttacccattcctgaaggacaaccgggaaaagatcgagaagatcctgaccttccgcatcccctactacgtgggccctctggccaggggaaacagcagattcgcctggatgaccagaaagagcgaggaaaccatcaccccctggaacttcgaggaagtggtggacaagggcgcttccgcccagagcttcatcgagcggatgaccaacttcgataagaacctgcccaacgagaaggtgctgcccaagcacagcctgctgtacgagtacttcaccgtgtataacgagctgaccaaagtgaaatacgtgaccgagggaatgagaaagcccgccttcctgagcggcgagcagaaaaaggccatcgtggacctgctgttcaagaccaaccggaaagtgaccgtgaagcagctgaaagaggactacttcaagaaaatcgagtgcttcgactccgtggaaatctccggcgtggaagatcggttcaacgcctccctgggcacataccacgatctgctgaaaattatcaaggacaaggacttcctggacaatgaggaaaacgaggacattctggaagatatcgtgctgaccctgacactgtttgaggacagagagatgatcgaggaacggctgaaaacctatgcccacctgttcgacgacaaagtgatgaagcagctgaagcggcggagatacaccggctggggcaggctgagccggaagctgatcaacggcatccgggacaagcagtccggcaagacaatcctggatttcctgaagtccgacggcttcgccaacagaaacttcatgcagctgatccacgacgacagcctgacctttaaagaggacatccagaaagcccaggtgtccggccagggcgatagcctgcacgagcacattgccaatctggccggcagccccgccattaagaagggcatcctgcagacagtgaaggtggtggacgagctcgtgaaagtgatgggccggcacaagcccgagaacatcgtgatcgaaatggccagagagaaccagaccacccagaagggacagaagaacagccgcgagagaatgaagcggatcgaagagggcatcaaagagctgggcagccagatcctgaaagaacaccccgtggaaaacacccagctgcagaacgagaagctgtacctgtactacctgcagaatgggcgggatatgtacgtggaccaggaactggacatcaaccggctgtccgactacgatgtggaccatatcgtgcctcagagctttctgaaggacgactccatcgacaacaaggtgctgaccagaagcgacaagaaccggggcaagagcgacaacgtgccctccgaagaggtcgtgaagaagatgaagaactactggcggcagctgctgaacgccaagctgattacccagagaaagttcgacaatctgaccaaggccgagagaggcggcctgagcgaactggataaggccggcttcatcaagagacagctggtggaaacccggcagatcacaaagcacgtggcacagatcctggactcccggatgaacactaagtacgacgagaatgacaagctgatccgggaagtgaaagtgatcaccctgaagtccaagctggtgtccgatttccggaaggatttccagttttacaaagtgcgcgagatcaacaactaccaccacgcccacgacgcctacctgaacgccgtcgtgggaaccgccctgatcaaaaagtaccctaagctggaaagcgagttcgtgtacggcgactacaaggtgtacgacgtgcggaagatgatcgccaagagcgagcaggaaatcggcaaggctaccgccaagtacttcttctacagcaacatcatgaactttttcaagaccgagattaccctggccaacggcgagatccggaagcggcctctgatcgagacaaacggcgaaaccggggagatcgtgtgggataagggccgggattttgccaccgtgcggaaagtgctgagcatgccccaagtgaatatcgtgaaaaagaccgaggtgcagacaggcggcttcagcaaagagtctatcctgcccaagaggaacagcgataagctgatcgccagaaagaaggactgggaccctaagaagtacggcggcttcgacagccccaccgtggcctattctgtgctggtggtggccaaagtggaaaagggcaagtccaagaaactgaagagtgtgaaagagctgctggggatcaccatcatggaaagaagcagcttcgagaagaatcccatcgactttctggaagccaagggctacaaagaagtgaaaaaggacctgatcatcaagctgcctaagtactccctgttcgagctggaaaacggccggaagagaatgctggcctctgccggcgaactgcagaagggaaacgaactggccctgccctccaaatatgtgaacttcctgtacctggccagccactatgagaagctgaagggctcccccgaggataatgagcagaaacagctgtttgtggaacagcacaagcactacctggacgagatcatcgagcagatcagcgagttctccaagagagtgatcctggccgacgctaatctggacaaagtgctgtccgcctacaacaagcaccgggataagcccatcagagagcaggccgagaatatcatccacctgtttaccctgaccaatctgggagcccctgccgccttcaagtactttgacaccaccatcgaccggaagaggtacaccagcaccaaagaggtgctggacgccaccctgatccaccagagcatcaccggcctgtacgagacacggatcgacctgtctcagctgggaggcgacaaaaggccggcggccacgaaaaaggccggccaggcaaaaaagaaaaagtaagaattcgcccttcttcgttgaacaacggaaactcgacttgccttccgcacaatacatcatttcttcttagctttttttcttcttcttcgttcatacagtttttttttgtttatcagcttacattttcttgaaccgtagctttcgttttcttctttttaactttccattcggagtttttgtatcttgtttcatagtttgtcccaggattagaatgattaggcatcgaaccttcaagaatttgattgaataaaacatcttcattcttaagatatgaagataatcttcaaaaggcccctgggaatctgaaagaagagaagcaggcccatttatatgggaaagaacaatagtatttcttatataggcccatttaagttgaaaacaatcttcaaaagtcccacatcgcttagataagaaaacgaagctgagtttatatacagctagagtcgaagtagtgattggttgaaccgcaaagtgggatgttttagagctagaaatagcaagttaaaataaggctagtccgttatcaacttgaaaaagtggcaccgagtcggtgcaacaaagcaccagtggtctagtggtagaatagtaccctgccacggtacagacccgggttcgattcccggctggtgcagatgctatagagagatctatgttttagagctagaaatagcaagttaaaataaggctagtccgttatcaacttgaaaaagtggcaccgagtcggtgcaacaaagcaccagtggtctagtggtagaatagtaccctgccacggtacagacccgggttcgattcccggctggtgcatgagcagaaagaagaagagagttttagagctagaaatagcaagttaaaataaggctagtccgttatcaacttgaaaaagtggcaccgagtcggtgcaacaaagcaccagtggtctagtggtagaatagtaccctgccacggtacagacccgggttcgattcccggctggtgcacgcttcagcatccttgtcgtgttttagagctagaaatagcaagttaaaataaggctagtccgttatcaacttgaaaaagtggcaccgagtcggtgcaacaaagcaccagtggtctagtggtagaatagtaccctgccacggtacagacccgggttcgattcccggctggtgcagcagatttggtatgatgtctgttttagagctagaaatagcaagttaaaataaggctagtccgttatcaacttgaaaaagtggcaccgagtcggtgcaacaaagcaccagtggtctagtggtagaatagtaccctgccacggtacagacccgggttcgattcccggctggtgcatggagctttatcctcgtatcgttttagagctagaaatagcaagttaaaataaggctagtccgttatcaacttgaaaaagtggcaccgagtcggtgctttttttctagagggcgaattcactggccgtcgttttacaacgtcgtgactgggaaaaccctggcgttacccaacttaatcgccttgcagcacatccccctttcgccagctggcgtaatagcgaagaggcccgcaccgatcgcccttcccaacagttgcgcagcctgaatggcgaatgctagagcagcttgagcttggatcagattgtcgtttcccgccttcagtttaaactatcagtgtttgacaggatatattggcgggtaaacctaagagaaaagagcgtttattagaataacggatatttaaaagggcgtgaaaaggtttatccgttcgtccatttgtatgtgcatgccaaccacagggttcccctcgggatcaaagtactttgatccaacccctccgctgctatagtgcagtcggcttctgacgttcagtgcagccgtcttctgaaaacgacatgtcgcacaagtcctaagttacgcgacaggctgccgccctgcccttttcctggcgttttcttgtcgcgtgttttagtcgcataaagtagaatacttgcgactagaaccggagacattacgccatgaacaagagcgccgccgctggcctgctgggctatgcccgcgtcagcaccgacgaccaggacttgaccaaccaacgggccgaactgcacgcggccggctgcaccaagctgttttccgagaagatcaccggcaccaggcgcgaccgcccggagctggccaggatgcttgaccacctacgccctggcgacgttgtgacagtgaccaggctagaccgcctggcccgcagcacccgcgacctactggacattgccgagcgcatccaggaggccggcgcgggcctgcgtagcctggcagagccgtgggccgacaccaccacgccggccggccgcatggtgttgaccgtgttcgccggcattgccgagttcgagcgttccctaatcatcgaccgcacccggagcgggcgcgaggccgccaaggcccgaggcgtgaagtttggcccccgccctaccctcaccccggcacagatcgcgcacgcccgcgagctgatcgaccaggaaggccgcaccgtgaaagaggcggctgcactgcttggcgtgcatcgctcgaccctgtaccgcgcacttgagcgcagcgaggaagtgacgcccaccgaggccaggcggcgcggtgccttccgtgaggacgcattgaccgaggccgacgccctggcggccgccgagaatgaacgccaagaggaacaagcatgaaaccgcaccaggacggccaggacgaaccgtttttcattaccgaagagatcgaggcggagatgatcgcggccgggtacgtgttcgagccgcccgcgcacgtctcaaccgtgcggctgcatgaaatcctggccggtttgtctgatgccaagctggcggcctggccggccagcttggccgctgaagaaaccgagcgccgccgtctaaaaaggtgatgtgtatttgagtaaaacagcttgcgtcatgcggtcgctgcgtatatgatgcgatgagtaaataaacaaatacgcaaggggaacgcatgaaggttatcgctgtacttaaccagaaaggcgggtcaggcaagacgaccatcgcaacccatctagcccgcgccctgcaactcgccggggccgatgttctgttagtcgattccgatccccagggcagtgcccgcgattgggcggccgtgcgggaagatcaaccgctaaccgttgtcggcatcgaccgcccgacgattgaccgcgacgtgaaggccatcggccggcgcgacttcgtagtgatcgacggagcgccccaggcggcggacttggctgtgtccgcgatcaaggcagccgacttcgtgctgattccggtgcagccaagcccttacgacatatgggccaccgccgacctggtggagctggttaagcagcgcattgaggtcacggatggaaggctacaagcggcctttgtcgtgtcgcgggcgatcaaaggcacgcgcatcggcggtgaggttgccgaggcgctggccgggtacgagctgcccattcttgagtcccgtatcacgcagcgcgtgagctacccaggcactgccgccgccggcacaaccgttcttgaatcagaacccgagggcgacgctgcccgcgaggtccaggcgctggccgctgaaattaaatcaaaactcatttgagttaatgaggtaaagagaaaatgagcaaaagcacaaacacgctaagtgccggccgtccgagcgcacgcagcagcaaggctgcaacgttggccagcctggcagacacgccagccatgaagcgggtcaactttcagttgccggcggaggatcacaccaagctgaagatgtacgcggtacgccaaggcaagaccattaccgagctgctatctgaatacatcgcgcagctaccagagtaaatgagcaaatgaataaatgagtagatgaattttagcggctaaaggaggcggcatggaaaatcaagaacaaccaggcaccgacgccgtggaatgccccatgtgtggaggaacgggcggttggccaggcgtaagcggctgggttgtctgccggccctgcaatggcactggaacccccaagcccgaggaatcggcgtgacggtcgcaaaccatccggcccggtacaaatcggcgcggcgctgggtgatgacctggtggagaagttgaaggccgcgcaggccgcccagcggcaacgcatcgaggcagaagcacgccccggtgaatcgtggcaagcggccgctgatcgaatccgcaaagaatcccggcaaccgccggcagccggtgcgccgtcgattaggaagccgcccaagggcgacgagcaaccagattttttcgttccgatgctctatgacgtgggcacccgcgatagtcgcagcatcatggacgtggccgttttccgtctgtcgaagcgtgaccgacgagctggcgaggtgatccgctacgagcttccagacgggcacgtagaggtttccgcagggccggccggcatggccagtgtgtgggattacgacctggtactgatggcggtttcccatctaaccgaatccatgaaccgataccgggaagggaagggagacaagcccggccgcgtgttccgtccacacgttgcggacgtactcaagttctgccggcgagccgatggcggaaagcagaaagacgacctggtagaaacctgcattcggttaaacaccacgcacgttgccatgcagcgtacgaagaaggccaagaacggccgcctggtgacggtatccgagggtgaagccttgattagccgctacaagatcgtaaagagcgaaaccgggcggccggagtacatcgagatcgagctagctgattggatgtaccgcgagatcacagaaggcaagaacccggacgtgctgacggttcaccccgattactttttgatcgatcccggcatcggccgttttctctaccgcctggcacgccgcgccgcaggcaaggcagaagccagatggttgttcaagacgatctacgaacgcagtggcagcgccggagagttcaagaagttctgtttcaccgtgcgcaagctgatcgggtcaaatgacctgccggagtacgatttgaaggaggaggcggggcaggctggcccgatcctagtcatgcgctaccgcaacctgatcgagggcgaagcatccgccggttcctaatgtacggagcagatgctagggcaaattgccctagcaggggaaaaaggtcgaaaagcactctttcctgtggatagcacgtacattgggaacccaaagccgtacattgggaaccggaacccgtacattgggaacccaaagccgtacattgggaaccggtcacacatgtaagtgactgatataaaagagaaaaaaggcgatttttccgcctaaaactctttaaaacttattaaaactcttaaaacccgcctggcctgtgcataactgtctggccagcgcacagccgaagagctgcaaaaagcgcctacccttcggtcgctgcgctccctacgccccgccgcttcgcgtcggcctatcgcggccgctggccgctcaaaaatggctggcctacggccaggcaatctaccagggcgcggacaagccgcgccgtcgccactcgaccgccggcgcccacatcaaggcaccctgcctcgcgcgtttcggtgatgacggtgaaaacctctgacacatgcagctcccggagacggtcacagcttgtctgtaagcggatgccgggagcagacaagcccgtcagggcgcgtcagcgggtgttggcgggtgtcggggcgcagccatgacccagtcacgtagcgatagcggagtgtatactggcttaactatgcggcatcagagcagattgtactgagagtgcaccatatgcggtgtgaaataccgcacagatgcgtaaggagaaaataccgcatcaggcgctcttccgcttcctcgctcactgactcgctgcgctcggtcgttcggctgcggcgagcggtatcagctcactcaaaggcggtaatacggttatccacagaatcaggggataacgcaggaaagaacatgtgagcaaaaggccagcaaaaggccaggaaccgtaaaaaggccgcgttgctggcgtttttccataggctccgcccccctgacgagcatcacaaaaatcgacgctcaagtcagaggtggcgaaacccgacaggactataaagataccaggcgtttccccctggaagctccctcgtgcgctctcctgttccgaccctgccgcttaccggatacctgtccgcctttctcccttcgggaagcgtggcgctttctcatagctcacgctgtaggtatctcagttcggtgtaggtcgttcgctccaagctgggctgtgtgcacgaaccccccgttcagcccgaccgctgcgccttatccggtaactatcgtcttgagtccaacccggtaagacacgacttatcgccactggcagcagccactggtaacaggattagcagagcgaggtatgtaggcggtgctacagagttcttgaagtggtggcctaactacggctacactagaaggacagtatttggtatctgcgctctgctgaagccagttaccttcggaaaaagagttggtagctcttgatccggcaaacaaaccaccgctggtagcggtggtttttttgtttgcaagcagcagattacgcgcagaaaaaaaggatctcaagaagatcctttgatcttttctacggggtctgacgctcagtggaacgaaaactcacgttaagggattttggtcatgcattctaggtactaaaacaattcatccagtaaaatataatattttattttctcccaatcaggcttgatccccagtaagtcaaaaaatagctcgacatactgttcttccccgatatcctccctgatcgaccggacgcagaaggcaatgtcataccacttgtccgccctgccgcttctcccaagatcaataaagccacttactttgccatctttcacaaagatgttgctgtctcccaggtcgccgtgggaaaagacaagttcctcttcgggcttttccgtctttaaaaaatcatacagctcgcgcggatctttaaatggagtgtcttcttcccagttttcgcaatccacatcggccagatcgttattcagtaagtaatccaattcggctaagcggctgtctaagctattcgtatagggacaatccgatatgtcgatggagtgaaagagcctgatgcactccgcatacagctcgataatcttttcagggctttgttcatcttcatactcttccgagcaaaggacgccatcggcctcactcatgagcagattgctccagccatcatgccgttcaaagtgcaggacctttggaacaggcagctttccttccagccatagcatcatgtccttttcccgttccacatcataggtggtccctttataccggctgtccgtcatttttaaatataggttttcattttctcccaccagcttatataccttagcaggagacattccttccgtatcttttacgcagcggtatttttcgatcagttttttcaattccggtgatattctcattttagccatttattatttccttcctcttttctacagtatttaaagataccccaagaagctaattataacaagacgaactccaattcactgttccttgcattctaaaaccttaaataccagaaaacagctttttcaaagttgttttcaaagttggcgtataacatagtatcgacggagccgattttgaaaccgcggtgatcacaggcagcaacgctctgtcatcgttacaatcaacatgctaccctccgcgagatcatccgtgtttcaaacccggcagcttagttgccgttcttccgaatagcatcggtaacatgagcaaagtctgccgccttacaacggctctcccgctgacgccgtcccggactgatgggctgcctgtatcgagtggtgattttgtgccgagctgccggtcggggagctgttggctggctggtggcaggatatattgtggtgtaaacaaattgacgcttagacaacttaataacacattgcggacgtttttaatgtactgaattaacgccgaattaattcgggggatctggattttagtactggattttggttttaggaattagaaattttattgatagaagtattttacaaatacaaatacatactaagggtttcttatatgctcaacacatgagcgaaaccctataggaaccctaattcccttatctgggaactactcacacattattatggagaaactcgagcttgtcgatcgacagatccggtcggcatctactctatttctttgccctcggacgagtgctggggcgtcggtttccactatcggcgagtacttctacacagccatcggtccagacggccgcgcttctgcgggcgatttgtgtacgcccgacagtcccggctccggatcggacgattgcgtcgcatcgaccctgcgcccaagctgcatcatcgaaattgccgtcaaccaagctctgatagagttggtcaagaccaatgcggagcatatacgcccggagtcgtggcgatcctgcaagctccggatgcctccgctcgaagtagcgcgtctgctgctccatacaagccaaccacggcctccagaagaagatgttggcgacctcgtattgggaatccccgaacatcgcctcgctccagtcaatgaccgctgttatgcggccattgtccgtcaggacattgttggagccgaaatccgcgtgcacgaggtgccggacttcggggcagtcctcggcccaaagcatcagctcatcgagagcctgcgcgacggacgcactgacggtgtcgtccatcacagtttgccagtgatacacatggggatcagcaatcgcgcatatgaaatcacgccatgtagtgtattgaccgattccttgcggtccgaatgggccgaacccgctcgtctggctaagatcggccgcagcgatcgcatccatagcctccgcgaccggttgtagaacagcgggcagttcggtttcaggcaggtcttgcaacgtgacaccctgtgcacggcgggagatgcaataggtcaggctctcgctaaactccccaatgtcaagcacttccggaatcgggagcgcggccgatgcaaagtgccgataaacataacgatctttgtagaaaccatcggcgcagctatttacccgcaggacatatccacgccctcctacatcgaagctgaaagcacgagattcttcgccctccgagagctgcatcaggtcggagacgctgtcgaacttttcgatcagaaacttctcgacagacgtcgcggtgagttcaggctttttcatatctcattgccccccgggatctgcgaaagctcgagagagatagatttgtagagagagactggtgatttcagcgtgtcctctccaaatgaaatgaacttccttatatagaggaaggtcttgcgaaggatagtgggattgtgcgtcatcccttacgtcagtggagatatcacatcaatccacttgctttgaagacgtggttggaacgtcttctttttccacgatgctcctcgtgggtgggggtccatctttgggaccactgtcggcagaggcatcttgaacgatagcctttcctttatcgcaatgatggcatttgtaggtgccaccttccttttctactgtccttttgatgaagtgacagatagctgggcaatggaatccgaggaggtttcccgatattaccctttgttgaaaagtctcaatagccctttggtcttctgagactgtatctttgatattcttggagtagacgagagtgtcgtgctccaccatgttatcacatcaatccacttgctttgaagacgtggttggaacgtcttctttttccacgatgctcctcgtgggtgggggtccatctttgggaccactgtcggcagaggcatcttgaacgatagcctttcctttatcgcaatgatggcatttgtaggtgccaccttccttttctactgtccttttgatgaagtgacagatagctgggcaatggaatccgaggaggtttcccgatattaccctttgttgaaaagtctcaatagccctttggtcttctgagactgtatctttgatattcttggagtagacgagagtgtcgtgctccaccatgttggcaagctgctctagccaatacgcaaaccgcctctccccgcgcgttggccgattcattaatgcagctggcacgacaggtttcccgactggaaagcgggcagtgagcgcaacgcaattaatgtgagttagctcactcattaggcaccccaggctttacactttatgcttccggctcgtatgttgtgtggaattgtgagcggataacaatttcacacaggaaacagctatgaccatgattacgcc

SEQ ID NO: 39 - DNA, 15734 bp, synthetic construct
  misc_feature 1..15734: note = nucleotides coding pNGPJ0014
  source 1..15734: mol_type = other DNA
aagcttgataatttatttgaaaattcataagaaaagcaaacgttacatgaattgatgaaacaatacaaagacagataaagccacgcacatttaggatattggccgagattactgaatattgagtaagatcacggaatttctgacaggagcatgtcttcaattcagcccaaatggcagttgaaatactcaaaccgccccatatgcaggagcggatcattcattgtttgtttggttgcctttgccaacatgggagtccaagattctgcagtcaaatctcggtgacgggcaggaccggacggggcggtaccggcaggctgaagtccagctgccagaaacccacgtcatgccagttcccgtgcttgaagccggccgcccgcagcatgccgcggggggcatatccgagcgcctcgtgcatgcgcacgctcgggtcgttgggcagcccgatgacagcgaccacgctcttgaagccctgtgcctccagggacttcagcaggtgggtgtagagcgtggagcccagtcccgtccgctggtggcggggggagacgtacacggtcgactcggccgtccagtcgtaggcgttgcgtgccttccaggggcccgcgtaggcgatgccggcgacctcgccgtccacctcggcgacgagccagggatagcgctcccgcagacggacgaggtcgtccgtccactcctgcggttcctgcggctcggtacggaagttgaccgtgcttgtctcgatgtagtggttgacgatggtgcagaccgccggcatgtccgcctcggtggcacggcggatgtcggccgggcgtcgttctgggctcatcgattcgatttggtgtatcgagattggttatgaaattcagatgctagtgtaatgtattggtaatttgggaagatataataggaagcaaggctatttatccatttctgaaaaggcgaaatggcgtcaccgcgagcgtcacgcgcattccgttcttgctgtaaagcgttgtttggtacacttttgactagcgaggcttggcgtgtcagcgtatctattcaaaagtcgttaatggctgcggatcaagaaaaagttggaatagaaacagaatacccgcgaaattcaggcccggttgccatgtcctacacgccgaaataaacgaccaaattagtagaaaaataaaaactgactcggatacttacgtcacgtcttgcgcactgatttgaaaaatctcagccatggctgcaggtcgacgagtcagtaataaacggcgtcaaagtggttgcagccggcacacacgagtcgtgtttatcaactcaaagcacaaatacttttcctcaacctaaaaataaggcaattagccaaaaacaactttgcgtgtaaacaacgctcaatacacgtgtcattttattattagctattgcttcaccgccttagctttctcgtgacctagtcgtcctcgtcttttcttcttcttcttctataaaacaatacccaaagagctcttcttcttcacaattcagatttcaatttctcaaaatcttaaaaactttctctcaattctctctaccgtgatcaaggtaaatttctgtgttccttattctctcaaaatcttcgattttgttttcgttcgatcccaatttcgtatatgttctttggtttagattctgttaatcttagatcgaagacgattttctgggtttgatcgttagatatcatcttaattctcgattagggtttcatagatatcatccgatttgttcaaataatttgagttttgtcgaataattactcttcgatttgtgatttctatctagatctggtgttagtttctagtttgtgcgatcgaatttgtcgattaatctgagtttttctgattaacagccatggactataaggaccacgacggagactacaaggatcatgatattgattacaaagacgatgacgataagatggccccaaagaagaagcggaaggtcggtatccacggagtcccagcagccgacaagaagtacagcatcggcctggacatcggcaccaactctgtgggctgggccgtgatcaccgacgagtacaaggtgcccagcaagaaattcaaggtgctgggcaacaccgaccggcacagcatcaagaagaacctgatcggagccctgctgttcgacagcggcgaaacagccgaggccacccggctgaagagaaccgccagaagaagatacaccagacggaagaaccggatctgctatctgcaagagatcttcagcaacgagatggccaaggtggacgacagcttcttccacagactggaagagtccttcctggtggaagaggataagaagcacgagcggcaccccatcttcggcaacatcgtggacgaggtggcctaccacgagaagtaccccaccatctaccacctgagaaagaaactggtggacagcaccgacaaggccgacctgcggctgatctatctggccctggcccacatgatcaagttccggggccacttcctgatcgagggcgacctgaaccccgacaacagcgacgtggacaagctgttcatccagctggtgcagacctacaaccagctgttcgaggaaaaccccatcaacgccagcggcgtggacgccaaggccatcctgtctgccagactgagcaagagcagacggctggaaaatctgatcgcccagctgcccggcgagaagaagaatggcctgttcggaaacctgattgccctgagcctgggcctgacccccaacttcaagagcaacttcgacctggccgaggatgccaaactgcagctgagcaaggacacctacgacgacgacctggacaacctgctggcccagatcggcgaccagtacgccgacctgtttctggccgccaagaacctgtccgacgccatcctgctgagcgacatcctgagagtgaacaccgagatcaccaaggcccccctgagcgcctctatgatcaagagatacgacgagcaccaccaggacctgaccctgctgaaagctctcgtgcggcagcagctgcctgagaagtacaaagagattttcttcgaccagagcaagaacggctacgccggctacattgacggcggagccagccaggaagagttctacaagttcatcaagcccatcctggaaaagatggacggcaccgaggaactgctcgtgaagctgaacagagaggacctgctgcggaagcagcggaccttcgacaacggcagcatcccccaccagatccacctgggagagctgcacgccattctgcggcggcaggaagatttttacccattcctgaaggacaaccgggaaaagatcgagaagatcctgaccttccgcatcccctactacgtgggccctctggccaggggaaacagcagattcgcctggatgaccagaaagagcgaggaaaccatcaccccctggaacttcgaggaagtggtggacaagggcgcttccgcccagagcttcatcgagcggatgaccaacttcgataagaacctgcccaacgagaaggtgctgcccaagcacagcctgctgtacgagtacttcaccgtgtataacgagctgaccaaagtgaaatacgtgaccgagggaatgagaaagcccgccttcctgagcggcgagcagaaaaaggccatcgtggacctgctgttcaagaccaaccggaaagtgaccgtgaagcagctgaaagaggactacttcaagaaaatcgagtgcttcgactccgtggaaatctccggcgtggaagatcggttcaacgcctccctgggcacataccacgatctgctgaaaattatcaaggacaaggacttcctggacaatgaggaaaacgaggacattctggaagatatcgtgctgaccctgacactgtttgaggacagagagatgatcgaggaacggctgaaaacctatgcccacctgttcgacgacaaagtgatgaagcagctgaagcggcggagatacaccggctggggcaggctgagccggaagctgatcaacggcatccgggacaagcagtccggcaagacaatcctggatttcctgaagtccgacggcttcgccaacagaaacttcatgcagctgatccacgacgacagcctgacctttaaagaggacatccagaaagcccaggtgtccggccagggcgatagcctgcacgagcacattgccaatctggccggcagccccgccattaagaagggcatcctgcagacagtgaaggtggtggacgagctcgtgaaagtgatgggccggcacaagcccgagaacatcgtgatcgaaatggccagagagaaccagaccacccagaagggacagaagaacagccgcgagagaatgaagcggatcgaagagggcatcaaagagctgggcagccagatcctgaaagaacaccccgtggaaaacacccagctgcagaacgagaagctgtacctgtactacctgcagaatgggcgggatatgtacgtggaccaggaactggacatcaaccggctgtccgactacgatgtggaccatatcgtgcctcagagctttctgaaggacgactccatcgacaacaaggtgctgaccagaagcgacaagaaccggggcaagagcgacaacgtgccctccgaagaggtcgtgaagaagatgaagaactactggcggcagctgctgaacgccaagctgattacccagagaaagttcgacaatctgaccaaggccgagagaggcggcctgagcgaactggataaggccggcttcatcaagagacagctggtggaaacccggcagatcacaaagcacgtggcacagatcctggactcccggatgaacactaagtacgacgagaatgacaagctgatccgggaagtgaaagtgatcaccctgaagtccaagctggtgtccgatttccggaaggatttccagttttacaaagtgcgcgagatcaacaactaccaccacgcccacgacgcctacctgaacgccgtcgtgggaaccgccctgatcaaaaagtaccctaagctggaaagcgagttcgtgtacggcgactacaaggtgtacgacgtgcggaagatgatcgccaagagcgagcaggaaatcggcaaggctaccgccaagtacttcttctacagcaacatcatgaactttttcaagaccgagattaccctggccaacggcgagatccggaagcggcctctgatcgagacaaacggcgaaaccggggagatcgtgtgggataagggccgggattttgccaccgtgcggaaagtgctgagcatgccccaagtgaatatcgtgaaaaagaccgaggtgcagacaggcggcttcagcaaagagtctatcctgcccaagaggaacagcgataagctgatcgccagaaagaaggactgggaccctaagaagtacggcggcttcgacagccccaccgtggcctattctgtgctggtggtggccaaagtggaaaagggcaagtccaagaaactgaagagtgtgaaagagctgctggggatcaccatcatggaaagaagcagcttcgagaagaatcccatcgactttctggaagccaagggctacaaagaagtgaaaaaggacctgatcatcaagctgcctaagtactccctgttcgagctggaaaacggccggaagagaatgctggcctctgccggcgaactgcagaagggaaacgaactggccctgccctccaaatatgtgaacttcctgtacctggccagccactatgagaagctgaagggctcccccgaggataatgagcagaaacagctgtttgtggaacagcacaagcactacctggacgagatcatcgagcagatcagcgagttctccaagagagtgatcctggccgacgctaatctggacaaagtgctgtccgcctacaacaagcaccgggataagcccatcagagagcaggccgagaatatcatccacctgtttaccctgaccaatctgggagcccctgccgccttcaagtactttgacaccaccatcgaccggaagaggtacaccagcaccaaagaggtgctggacgccaccctgatccaccagagcatcaccggcctgtacgagacacggatcgacctgtctcagctgggaggcgacaaaaggccggcggccacgaaaaaggccggccaggcaaaaaagaaaaagtaagaattcgcccttcttcgttgaacaacggaaactcgacttgccttccgcacaatacatcatttcttcttagctttttttcttcttcttcgttcatacagtttttttttgtttatcagcttacattttcttgaaccgtagctttcgttttcttctttttaactttccattcggagtttttgtatcttgtttcatagtttgtcccaggattagaatgattaggcatcgaaccttcaagaatttgattgaataaaacatcttcattcttaagatatgaagataatcttcaaaaggcccctgggaatctgaaagaagagaagcaggcccatttatatgggaaagaacaatagtatttcttatataggcccatttaagttgaaaacaatcttcaaaagtcccacatcgcttagataagaaaacgaagctgagtttatatacagctagagtcgaagtagtgattgtgagaccgagagagtcatcgagggtgatctcaaccctgataactctgatgtggataagttgttcatccagctcgtgcagacctacaaccagcttttcgaagagaaccctatcaacgctggtctcagttttagagctagaaatagcaagttaaaataaggctagtccgttatcaacttgaaaaagtggcaccgagtcggtgctttttttctagagggcgaattcactggccgtcgttttacactggccgtcgttttacaacgtcgtgactgggaaaaccctggcgttacccaacttaatcgccttgcagcacatccccctttcgccagctggcgtaatagcgaagaggcccgcaccgatcgcccttcccaacagttgcgcagcctgaatggcgaatgctagagcagcttgagcttggatcagattgtcgtttcccgccttcagtttaaactatcagtgtttgacaggatatattggcgggtaaacctaagagaaaagagcgtttattagaataacggatatttaaaagggcgtgaaaaggtttatccgttcgtccatttgtatgtgcatgccaaccacagggttcccctcgggatcaaagtactttgatccaacccctccgctgctatagtgcagtcggcttctgacgttcagtgcagccgtcttctgaaaacgacatgtcgcacaagtcctaagttacgcgacaggctgccgccctgcccttttcctggcgttttcttgtcgcgtgttttagtcgcataaagtagaatacttgcgactagaaccggagacattacgccatgaacaagagcgccgccgctggcctgctgggctatgcccgcgtcagcaccgacgaccaggacttgaccaaccaacgggccgaactgcacgcggccggctgcaccaagctgttttccgagaagatcaccggcaccaggcgcgaccgcccggagctggccaggatgcttgaccacctacgccctggcgacgttgtgacagtgaccaggctagaccgcctggcccgcagcacccgcgacctactggacattgccgagcgcatccaggaggccggcgcgggcctgcgtagcctggcagagccgtgggccgacaccaccacgccggccggccgcatggtgttgaccgtgttcgccggcattgccgagttcgagcgttccctaatcatcgaccgcacccggagcgggcgcgaggccgccaaggcccgaggcgtgaagtttggcccccgccctaccctcaccccggcacagatcgcgcacgcccgcgagctgatcgaccaggaaggccgcaccgtgaaagaggcggctgcactgcttggcgtgcatcgctcgaccctgtaccgcgcacttgagcgcagcgaggaagtgacgcccaccgaggccaggcggcgcggtgccttccgtgaggacgcattgaccgaggccgacgccctggcggccgccgagaatgaacgccaagaggaacaagcatgaaaccgcaccaggacggccaggacgaaccgtttttcattaccgaagagatcgaggcggagatgatcgcggccgggtacgtgttcgagccgcccgcgcacgtctcaaccgtgcggctgcatgaaatcctggccggtttgtctgatgccaagctggcggcctggccggccagcttggccgctgaagaaaccgagcgccgccgtctaaaaaggtgatgtgtatttgagtaaaacagcttgcgtcatgcggtcgctgcgtatatgatgcgatgagtaaataaacaaatacgcaaggggaacgcatgaaggttatcgctgtacttaaccagaaaggcgggtcaggcaagacgaccatcgcaacccatctagcccgcgccctgcaactcgccggggccgatgttctgttagtcgattccgatccccagggcagtgcccgcgattgggcggccgtgcgggaagatcaaccgctaaccgttgtcggcatcgaccgcccgacgattgaccgcgacgtgaaggccatcggccggcgcgacttcgtagtgatcgacggagcgccccaggcggcggacttggctgtgtccgcgatcaaggcagccgacttcgtgctgattccggtgcagccaagcccttacgacatatgggccaccgccgacctggtggagctggttaagcagcgcattgaggtcacggatggaaggctacaagcggcctttgtcgtgtcgcgggcgatcaaaggcacgcgcatcggcggtgaggttgccgaggcgctggccgggtacgagctgcccattcttgagtcccgtatcacgcagcgcgtgagctacccaggcactgccgccgccggcacaaccgttcttgaatcagaacccgagggcgacgctgcccgcgaggtccaggcgctggccgctgaaattaaatcaaaactcatttgagttaatgaggtaaagagaaaatgagcaaaagcacaaacacgctaagtgccggccgtccgagcgcacgcagcagcaaggctgcaacgttggccagcctggcagacacgccagccatgaagcgggtcaactttcagttgccggcggaggatcacaccaagctgaagatgtacgcggtacgccaaggcaagaccattaccgagctgctatctgaatacatcgcgcagctaccagagtaaatgagcaaatgaataaatgagtagatgaattttagcggctaaaggaggcggcatggaaaatcaagaacaaccaggcaccgacgccgtggaatgccccatgtgtggaggaacgggcggttggccaggcgtaagcggctgggttgtctgccggccctgcaatggcactggaacccccaagcccgaggaatcggcgtgacggtcgcaaaccatccggcccggtacaaatcggcgcggcgctgggtgatgacctggtggagaagttgaaggccgcgcaggccgcccagcggcaacgcatcgaggcagaagcacgccccggtgaatcgtggcaagcggccgctgatcgaatccgcaaagaatcccggcaaccgccggcagccggtgcgccgtcgattaggaagccgcccaagggcgacgagcaaccagattttttcgttccgatgctctatgacgtgggcacccgcgatagtcgcagcatcatggacgtggccgttttccgtctgtcgaagcgtgaccgacgagctggcgaggtgatccgctacgagcttccagacgggcacgtagaggtttccgcagggccggccggcatggccagtgtgtgggattacgacctggtactgatggcggtttcccatctaaccgaatccatgaaccgataccgggaagggaagggagacaagcccggccgcgtgttccgtccacacgttgcggacgtactcaagttctgccggcgagccgatggcggaaagcagaaagacgacctggtagaaacctgcattcggttaaacaccacgcacgttgccatgcagcgtacgaagaaggccaagaacggccgcctggtgacggtatccgagggtgaagccttgattagccgctacaagatcgtaaagagcgaaaccgggcggccggagtacatcgagatcgagctagctgattggatgtaccgcgagatcacagaaggcaagaacccggacgtgctgacggttcaccccgattactttttgatcgatcccggcatcggccgttttctctaccgcctggcacgccgcgccgcaggcaaggcagaagccagatggttgttcaagacgatctacgaacgcagtggcagcgccggagagttcaagaagttctgtttcaccgtgcgcaagctgatcgggtcaaatgacctgccggagtacgatttgaaggaggaggcggggcaggctggcccgatcctagtcatgcgctaccgcaacctgatcgagggcgaagcatccgccggttcctaatgtacggagcagatgctagggcaaattgccctagcaggggaaaaaggtcgaaaagcactctttcctgtggatagcacgtacattgggaacccaaagccgtacattgggaaccggaacccgtacattgggaacccaaagccgtacattgggaaccggtcacacatgtaagtgactgatataaaagagaaaaaaggcgatttttccgcctaaaactctttaaaacttattaaaactcttaaaacccgcctggcctgtgcataactgtctggccagcgcacagccgaagagctgcaaaaagcgcctacccttcggtcgctgcgctccctacgccccgccgcttcgcgtcggcctatcgcggccgctggccgctcaaaaatggctggcctacggccaggcaatctaccagggcgcggacaagccgcgccgtcgccactcgaccgccggcgcccacatcaaggcaccctgcctcgcgcgtttcggtgatgacggtgaaaacctctgacacatgcagctcccggagacggtcacagcttgtctgtaagcggatgccgggagcagacaagcccgtcagggcgcgtcagcgggtgttggcgggtgtcggggcgcagccatgacccagtcacgtagcgatagcggagtgtatactggcttaactatgcggcatcagagcagattgtactgagagtgcaccatatgcggtgtgaaataccgcacagatgcgtaaggagaaaataccgcatcaggcgctcttccgcttcctcgctcactgactcgctgcgctcggtcgttcggctgcggcgagcggtatcagctcactcaaaggcggtaatacggttatccacagaatcaggggataacgcaggaaagaacatgtgagcaaaaggccagcaaaaggccaggaaccgtaaaaaggccgcgttgctggcgtttttccataggctccgcccccctgacgagcatcacaaaaatcgacgctcaagtcagaggtggcgaaacccgacaggactataaagataccaggcgtttccccctggaagctccctcgtgcgctctcctgttccgaccctgccgcttaccggatacctgtccgcctttctcccttcgggaagcgtggcgctttctcatagctcacgctgtaggtatctcagttcggtgtaggtcgttcgctccaagctgggctgtgtgcacgaaccccccgttcagcccgaccgctgcgccttatccggtaactatcgtcttgagtccaacccggtaagacacgacttatcgccactggcagcagccactggtaacaggattagcagagcgaggtatgtaggcggtgctacagagttcttgaagtggtggcctaactacggctacactagaaggacagtatttggtatctgcgctctgctgaagccagttaccttcggaaaaagagttggtagctcttgatccggcaaacaaaccaccgctggtagcggtggtttttttgtttgcaagcagcagattacgcgcagaaaaaaaggatctcaagaagatcctttgatcttttctacggggtctgacgctcagtggaacgaaaactcacgttaagggattttggtcatgcattctaggtactaaaacaattcatccagtaaaatataatattttattttctcccaatcaggcttgatccccagtaagtcaaaaaatagctcgacatactgttcttccccgatatcctccctgatcgaccggacgcagaaggcaatgtcataccacttgtccgccctgccgcttctcccaagatcaataaagccacttactttgccatctttcacaaagatgttgctgtctcccaggtcgccgtgggaaaagacaagttcctcttcgggcttttccgtctttaaaaaatcatacagctcgcgcggatctttaaatggagtgtcttcttcccagttttcgcaatccacatcggccagatcgttattcagtaagtaatccaattcggctaagcggctgtctaagctattcgtatagggacaatccgatatgtcgatggagtgaaagagcctgatgcactccgcatacagctcgataatcttttcagggctttgttcatcttcatactcttccgagcaaaggacgccatcggcctcactcatgagcagattgctccagccatcatgccgttcaaagtgcaggacctttggaacaggcagctttccttccagccatagcatcatgtccttttcccgttccacatcataggtggtccctttataccggctgtccgtcatttttaaatataggttttcattttctcccaccagcttatataccttagcaggagacattccttccgtatcttttacgcagcggtatttttcgatcagttttttcaattccggtgatattctcattttagccatttattatttccttcctcttttctacagtatttaaagataccccaagaagctaattataacaagacgaactccaattcactgttccttgcattctaaaaccttaaataccagaaaacagctttttcaaagttgttttcaaagttggcgtataacatagtatcgacggagccgattttgaaaccgcggtgatcacaggcagcaacgctctgtcatcgttacaatcaacatgctaccctccgcgagatcatccgtgtttcaaacccggcagcttagttgccgttcttccgaatagcatcggtaacatgagcaaagtctgccgccttacaacggctctcccgctgacgccgtcccggactgatgggctgcctgtatcgagtggtgattttgtgccgagctgccggtcggggagctgttggctggctggtggcaggatatattgtggtgtaaacaaattgacgcttagacaacttaataacacattgcggacgtttttaatgtactgaattaacgccgaattaattcgggggatctggattttagtactggattttggttttaggaattagaaattttattgatagaagtattttacaaatacaaatacatactaagggtttcttatatgctcaacacatgagcgaaaccctataggaaccctaattcccttatctgggaactactcacacattattatggagaaactcgagcttgtcgatcgacagatccggtcggcatctactctatttctttgccctcggacgagtgctggggcgtcggtttccactatcggcgagtacttctacacagccatcggtccagacggccgcgcttctgcgggcgatttgtgtacgcccgacagtcccggctccggatcggacgattgcgtcgcatcgaccctgcgcccaagctgcatcatcgaaattgccgtcaaccaagctctgatagagttggtcaagaccaatgcggagcatatacgcccggagtcgtggcgatcctgcaagctccggatgcctccgctcgaagtagcgcgtctgctgctccatacaagccaaccacggcctccagaagaagatgttggcgacctcgtattgggaatccccgaacatcgcctcgctccagtcaatgaccgctgttatgcggccattgtccgtcaggacattgttggagccgaaatccgcgtgcacgaggtgccggacttcggggcagtcctcggcccaaagcatcagctcatcgagagcctgcgcgacggacgcactgacggtgtcgtccatcacagtttgccagtgatacacatggggatcagcaatcgcgcatatgaaatcacgccatgtagtgtattgaccgattccttgcggtccgaatgggccgaacccgctcgtctggctaagatcggccgcagcgatcgcatccatagcctccgcgaccggttgtagaacagcgggcagttcggtttcaggcaggtcttgcaacgtgacaccctgtgcacggcgggagatgcaataggtcaggctctcgctaaactccccaatgtcaagcacttccggaatcgggagcgcggccgatgcaaagtgccgataaacataacgatctttgtagaaaccatcggcgcagctatttacccgcaggacatatccacgccctcctacatcgaagctgaaagcacgagattcttcgccctccgagagctgcatcaggtcggagacgctgtcgaacttttcgatcagaaacttctcgacagacgtcgcggtgagttcaggctttttcatatctcattgccccccgggatctgcgaaagctcgagagagatagatttgtagagagagactggtgatttcagcgtgtcctctccaaatgaaatgaacttccttatatagaggaaggtcttgcgaaggatagtgggattgtgcgtcatcccttacgtcagtggagatatcacatcaatccacttgctttgaagacgtggttggaacgtcttctttttccacgatgctcctcgtgggtgggggtccatctttgggaccactgtcggcagaggcatcttgaacgatagcctttcctttatcgcaatgatggcatttgtaggtgccaccttccttttctactgtccttttgatgaagtgacagatagctgggcaatggaatccgaggaggtttcccgatattaccctttgttgaaaagtctcaatagccctttggtcttctgagactgtatctttgatattcttggagtagacgagagtgtcgtgctccaccatgttatcacatcaatccacttgctttgaagacgtggttggaacgtcttctttttccacgatgctcctcgtgggtgggggtccatctttgggaccactgtcggcagaggcatcttgaacgatagcctttcctttatcgcaatgatggcatttgtaggtgccaccttccttttctactgtccttttgatgaagtgacagatagctgggcaatggaatccgaggaggtttcccgatattaccctttgttgaaaagtctcaatagccctttggtcttctgagactgtatctttgatattcttggagtagacgagagtgtcgtgctccaccatgttggcaagctgctctagccaatacgcaaaccgcctctccccgcgcgttggccgattcattaatgcagctggcacgacaggtttcccgactggaaagcgggcagtgagcgcaacgcaattaatgtgagttagctcactcattaggcaccccaggctttacactttatgcttccggctcgtatgttgtgtggaattgtgagcggataacaatttcacacaggaaacagctatgaccatgattacgcc

SEQ ID NO: 40 - DNA, 92 bp, synthetic construct
  source 1..92: mol_type = other DNA
  misc_feature 1..92: note = exon 1 of DWF5-1
atggtggagaacaagttggtacactctccattaatcacttatggatcaatgctcagtcttctatctttcacaccaccttttgtaatcctcat

SEQ ID NO: 41 - DNA, 223 bp, synthetic construct
  source 1..223: mol_type = other DNA
  misc_feature 1..223: note = exon 2 of DWF5-1
gtggtatacaaatgtgcacgctgatgggtctatcttgaaaacgttcaatcatctaagggaaaatggtttgcaaggattaattgatatttggccaaaacctactgcaattgctgggaagctaatcatttgttatgctctatttgaggcggcactacagcttctattgcctggtaaaacagtcgaaggcccaatatctccaactggacataggcctgtctataag

SEQ ID NO: 42 - DNA, 56 bp, synthetic construct
  source 1..56: mol_type = other DNA
  misc_feature 1..56: note = exon 3 of DWF5-1
gctaatggcatggcagcatatgcagtgacactgatcacatatatcagtctctggtg

SEQ ID NO: 43 - DNA, 103 bp, synthetic construct
  source 1..103: mol_type = other DNA
  misc_feature 1..103: note = exon 4 of DWF5-1
gtttggaatatttaatcctgcaattgtttatgaccatctgggcgagattttctctacacttatttttgggagtttagtcttctgtgttttattgtacattaaa

SEQ ID NO: 44 - DNA, 66 bp, synthetic construct
  source 1..66: mol_type = other DNA
  misc_feature 1..66: note = exon 5 of DWF5-1
ggtcatgttgcaccatcttccactgattccggctcatcagggaacataatagttgacttctattgg

SEQ ID NO: 45 - DNA, 114 bp, synthetic construct; identical to SEQ ID NO: 9
  source 1..114: mol_type = other DNA
  misc_feature 1..114: note = exon 6 of DWF5-1

SEQ ID NO: 46 - DNA, 127 bp, synthetic construct; identical to SEQ ID NO: 10
  source 1..127: mol_type = other DNA
  misc_feature 1..127: note = exon 7 of DWF5-1

SEQ ID NO: 47 - DNA, 126 bp, synthetic construct; identical to SEQ ID NO: 11
  source 1..126: mol_type = other DNA
  misc_feature 1..126: note = exon 8 of DWF5-1

SEQ ID NO: 48 - DNA, 65 bp, synthetic construct; identical to SEQ ID NO: 12
  source 1..65: mol_type = other DNA
  misc_feature 1..65: note = exon 9 of DWF5-1

SEQ ID NO: 49 - DNA, 82 bp, synthetic construct; identical to SEQ ID NO: 13
  source 1..82: mol_type = other DNA
  misc_feature 1..82: note = exon 10 of DWF5-1

SEQ ID NO: 50 - DNA, 83 bp, synthetic construct
  source 1..83: mol_type = other DNA
  misc_feature 1..83: note = exon 11 of DWF5-1
ttcattccctacttctacgtcatctttctaataatcctccttctcgatcgagctaaaagggacgatgaccgatgcaaggcaaa

SEQ ID NO: 51 - DNA, 67 bp, synthetic construct
  source 1..67: mol_type = other DNA
  misc_feature 1..67: note = exon 12 of DWF5-1
gtatggcaagtactggaaattgtattgtgaaaaggttccttacagagttatcccaggaatttactag

SEQ ID NO: 52 - DNA, 1040 bp, synthetic construct
  source 1..1040: mol_type = other DNA
  misc_feature 1..1040: note = intron 1 of DWF5-1
gtaagtccaacacccacttttcatattgatctatttttgttgattttattgtcttttcttgttttggggtttttgttttcttgtgtaaaagttcagatctttgaatgggttgttgtatcatgagttaaagattggatcttttttttttttttttgtttagttttggtttgatttgcttgctatagtttaactgtcttctagttataaaaatgttttttttttggtgtaattgagattcattattatttagctctaaagaagcaagtgttttctagttataaaaatgtttgttttttgggtgtaattgagattcattattatttagctctaaagaagcaagtgtttggttagagttatgcttgtatttgtttgctaactaaacatggtaatacttgtgcatgatttaatacctgtgccccctttttgatttgggaggtctaaaagagagacactagagtggatgaagtttttcttttgaaggggatgaaaagtagaaataggaataacaggttgctccaataagtgtagattctaattttagctaatatcaattgatgatggactacgtttcaatcccgaatgagtttgattcggttaaataaagcacatgcatctgttatgctccaccttttaagttttcaaaggattcacaatcaatagactattttttactagtagtctacctactgcagccccatcttttatggggttatggtacacatttgctgagtcataattttagttagtatgatcttgaaatgtggttctgtggttctttccgtagacattcgttaattggcctatacagaaaatgatttgcatttagtcatgtgaaaggagtaaaaatgctatgtaaataaaaaattacaaattgatcctgctgtaaattttttgaatgtttcaccagtaacagatgatttctgctgccttagccacagatctttccactgtgttatgtacagtagctcaaaagtgtcttgatgaggaaatgtaattgtataactgcactaatttttggaccttaatgggcctacttgcag

SEQ ID NO: 53 - DNA, 177 bp, synthetic construct
  source 1..177: mol_type = other DNA
  misc_feature 1..177: note = intron 2 of DWF5-1
gtatatggcagttatgctatacacaagtacagtgtgcatcttgcatttatagtttgtgtaatttgtcttagttgagtttatttcaagtgatgcaatggttgatgtgctatgatctgtctttcctctgttcattgtacaactgtataacttgcctcttatatcctctacttattgcag

SEQ ID NO: 54 - DNA, 832 bp, synthetic construct
  source 1..832: mol_type = other DNA
  misc_feature 1..832: note = intron 3 of DWF5-1
gtagggatttcatcaatttttgctttttgactagcttgctgaatcttgagacctcgattctttatgtattggttcgttaatctcacttgccagcttcagcttgacaatgcttgggacagcattggggtcttggggacatgaatttcatcaagggaatctaaaaaaaatatgctcttttgtgtttagggcttcaacaatttgtattaaactgataaaaagttttttcacctaaacaaacaccaatcaattcgtccaaatattaatggacactaaagaatacaacaaaaataatgaattggtgcacttttaaggtcaacgtacactctatcctccccagacccttgtgttattgctattgttgttgttgttttgtatagtgtatttattgatattgtgtgactgtctctttcaaaagtttgtagagatggcatacttgtatttacttaatatgtcttcaactcgcttcctagcaggtctagttttttccatgggccaaacacatgaatttgttttatgatgggtggttgtaagacttgaatccaaaacctttgcttgctctaataccgtatccaaaaaaaataaaataaaccttaggcctaaataaaccgaaagttagcatatttaaggaatatccaagataatataaggagataacatcacattgtctcaacgtatatgagacactctaacaactcctgacgtccagaacctttacttgtttgattgttcattttatctatgagctattgtttgtgagaaaggtgcatattatggtccattaaactcatcagttcactctctctagttatgtttttttttccgtgtctttcag

SEQ ID NO: 55 - DNA, 99 bp, synthetic construct
  source 1..99: mol_type = other DNA
  misc_feature 1..99: note = intron 4 of DWF5-1
gtaagtattttaagtaccctcagtacacctcttatctctgattctttgcttagtattatacctgtctgacaccttgtgctgacatttataatttataag

SEQ ID NO: 56 - DNA, 179 bp, synthetic construct
  source 1..179: mol_type = other DNA
  misc_feature 1..179: note = intron 5 of DWF5-1
gtaagcatcttttgaaaatttaactgtgaacttcactacttcattttgtgtctttataggaaaaataagcatgatgatgttataccacaaattaagtcaaggaagtcaatatctagtacttgcatcatctctggagttgaaagtgatgtcataatttatgacctgatgaactctttcag

SEQ ID NO: 57 - DNA, 683 bp, synthetic construct
  source 1..683: mol_type = other DNA
  misc_feature 1..683: note = intron 6 of DWF5-1
gtaaatgatgtaatgaagtccttgatagtgagaattaaaactttcccaatatttctcggtcctattgttcctgagttggtgaattttacaagcccttttattggggatcccttgccagttgttcagtttttaggtcatgcaagtaagaaaatgatataatattcatttgcttccgtcaatagatgtttaacaggataagaaaaagacattttcttataccatttaatggaaaaaaacagtggactgttatctaaagtactccctccgttccaatttatttgaccaattttgacttggcatggagtttaagaaagtaaagaagacttgaattttgtggtcttaaactaaaggtatgtcaaatgtaccaaaaatgcctcggggtcttaaacatgccatgtggaaagttgaaattaagagttgctaaaaaaagaaagaatcattctttttgaaatggactaaaaaggaaagcaggccaaacaaattgagaaggagggagtaattatgtttacttgacatgaccctatcacagcttaggtgtctttactttgtgctcgttctttcaccttgacccctaacattctttacctggatttcagttgattgtcaatagaaaaacctagtatatgaacttcattttgatgtttgacagtcgatagtttgtataacatattcttacttttcag

SEQ ID NO: 58 - DNA, 2718 bp, synthetic construct
  source 1..2718: mol_type = other DNA
  misc_feature 1..2718: note = intron 7 of DWF5-1
gtttgtgcatactgtgttttctatattgatatagcaagtaccttcccagtgctctgattgcaaatgctgacatttcttgtttctctatttcggtggacgcctatatataatcttctctggatctcaaattcgtttggcagctggcttttatatatgttggggatgcttggtgtgggttccaagcatatatacgtctcctggaatgtatcttgttaaacaacctgtgaatcttgggcttcaggtatttttgcatccaagaagaatttgctaaatgcatataaaatataaagttattgccaataagcattacttactgtttatttttatactcaactactattttgggatttgtacttagtttttacttagtcttcgtcttctatttgataaccaagaaatccccgagggctggtggggtacagttcgaagctcaatggataataagctcattcctcttcccttctccacttaattaccaggctattgtctgtggcaagtttctaatatatggcaaatacatatctgcagcctgcatatcatgtgcttggtcttcatctttatcaacttatttgaagaaatgttcttagtgaaccatattcacctctagttcatgcactgaaatactcaatcacgagtcacggcccacaatgtggttataatcagtgctatttatccagcttgtgagatcagatcgactactctactaccatcattccattgcctagcacgaaaggttgcttaggacaaattatggaaaatgttctttgcagtaataccaagaaagtagtagctcactgtgaaagtttcactcaaataatgttgctgaaggtgaaaggttcaaaaaaggcatcatatttctgctgaactgaaatctcctcacagtctggctttgtaacttttgtagacatataattgtaattcaaaaacacttttaaatcgaatgaacttaaggcaataatgaagagtgaaaatgagggtgactgttgagcatatggtagagagtacaaaccatgatagataacagaagatagatatcttccaaactccctgatagagtcagaagttgtggattattagtttcaagcttgagaaaacccctggagatgtgaaataatgtacttagaatatcttccaatcgacatttatccctttaaagtatgacggaagtcccattgctggcagaatcatctgtagcataacagataatatgagcaaatgagaccattcagccattcatcaatggctaacgtgttcatttttcgccaagctagcatttcttttgttgcatggatgtgtaatttttctcctttgtttcattttctttgacattttcacttttcagggtgtccattactctcttcaacattggctttattgcttcctctgttctaattgatatgacactcttttcactatgaagttgtcagatattttccaccagtctaacagtatttctcaatgactattgcttaacctcttaaaaataactgtggtttttctcgactatactattttttcgattggtttgacaatactatttactcttttgatcattcctttgatattttattcgattagcactataggtatggaaaaattaaaatactacattcaaatgtcatataaaattagaggaaaggagtatataagtttttagtcaaagagttggtaatttgtataattttatttaaaatgataatgttcgatattagaacattgagtcaaccttcttaagaggaagtacaatctgggttcgttagagtacttcagatgagttgcatcctatattttcgatgatatcttccatttctggtattttaaacgatcatgtaaagaaaaaacagaacacattcttgaattgtcaaatgaccaagaaaggttctgtattgagtgttcacttttaccaatagggtctacccttgggatgatggtgtttcacttttaaattccctgagaattgcgaccttttgcccccacccaacacaccttaggacattttagatcagtgtatgtagaatttacctgtccctattggtagcaacatacgttttacggttagaaatttgactatccaatgttatagtttcttatttgccatcagggcatgtgatattttgaaacttccgttacttcaatccactataaaaaaactacacgtattaacatggcttgtagagcgcacacattcatttgctaatagcgacataagtatctgaaaaggagagaattatgagtacaattacttccctaatgtttcatccaacttattgaccttcactagattttacaacttggatggtggatgtacttcatagtacatacggattgtttcgttagttttcacatgtttcatttgatgtattataaatgttctgcataacagaaaaacaagacttattctagaattgtctgatgaagcagagaaaggttgctgattttttttgtcaactaggggtcttcccttggggacaatggtctttcacgtgatctctctgagaattgcaatgatttgcgacgatgcaccagtttgccattttgtcattgcaaggcaaatttttggctagaaaacattgagtgataatgtgttatctgaaattgatcattggtgcattgcatcaacctgcttaaggaaaccacatgtagtaaaatgacttggagagcatatgcaattttattgctttcggtttctaacgaggaaagttctttctgttatttcag

SEQ ID NO: 59 - DNA, 87 bp, synthetic construct
  source 1..87: mol_type = other DNA
  misc_feature 1..87: note = intron 8 of DWF5-1
gtcaaatgataccatctgtgaatttatttttcgaactctcttacccttatttgatgatttttgacttggttccttcactcaatgcag

SEQ ID NO: 60 - DNA, 1133 bp, synthetic construct
  source 1..1133: mol_type = other DNA
  misc_feature 1..1133: note = intron 9 of DWF5-1
gtcagttcctttctttgttctcctgctgacgttttacttctgcaatttagacactacaacagtttttttggggggaggtaataattgtatcaaattcagcactaagaaagtgctgcagaagtatatccatcagtagtcaaatccagcagttaagaatgtattctaatcctagtcttgtagggattctataagatctaaaactgttcatcatctttcattattctttgcaccaaaaaacaaaataacaaactacagatcattttgatctttttggatggaacttggtttgccttcaaaacatcttttccttcctctcccaattgtccaccaaacgcaagcaaggatggcatttcaccattttgtttggctttattcgtgcctgatttattccagctacttagtagatcattgtgattgctaggcatcatccattgaagtcccactatgtttaggaataaatgccatagctgattagtcatttgacagtgcaaaaatagatagtaatagtttctgacctttctccacacaaaaaacattttgtacaaaagtataatgcccctcttctgttaagttctcttgagtttgacttgcttccatagtcatcaagtcagtcaccatgtgaaacatgcaactttgtatggagtttttttctccatatcttcttccacggccagcacctgttccgttgagcattaatcatcagtcttgtagcatgagtagaccgtaaaggaagcaatgcttgtggcatccatattgctctttcttcataactggacagttctggagcatgctctaatgcatcaatcaatcaactattctagttagttctcagtcatttagcttactcctaaattgtgtactggattgtaaaactacgaaattgtattgttattctcctatattaccagtctcattcttatagaggctgtacttgattgcattaacaaggaattctgaataaataccttctatatttctaagaaaagcatctagaatttattctacttttcttatatcccgttttctaacgccaaacaaattcatatattgatgtataatacatgtcaattattttgcttatagcggcttgagacatcatacaatttacataatatgtttaaaccattttgcag

SEQ ID NO: 61 - DNA, 159 bp, synthetic construct
  source 1..159: mol_type = other DNA
  misc_feature 1..159: note = intron 10 of DWF5-1
gtaagcgttcatttacatcattactctgtatttttcttctttccgtattagagagaattccataatcaattttatctttcttgaattttgcattttgttcttgacattgctgaaatctaacatcctgtcccccttctttactttttcttgtacttgcag

SEQ ID NO: 62 - DNA, 601 bp, synthetic construct
  source 1..601: mol_type = other DNA
  misc_feature 1..601: note = intron 11 of DWF5-1
gtaagaaagcacacaccctcatttttacctggatttttcatatggttctccactcctcactaataaactcgatcaaattgattagtaatagtcatacatgtcttgctggttgtgttgttaacaagacttgagaacttatcgatttctttgctcatggacagaataaacttatgatatcctcaaaataattatcctggcattccgccacccccatggcataatagatccctagaggtggcacctgagggtgtgacctagacgtcaatgaaatgattgacaatcatgggattaggggttcaaatcccaatcgaagacaaaaacttaggtgatttttaccccatttgcctagaccttaacaggcagagtagtcagtatatgtgttggtaggagttaacacgtagcaggtagagtgtagctgaaatggacgaaagctggcctagacaccactgttttttagaaaaaactagttgagtagccgaaggtcgtcttgatctgtccctaaagatcgttacgaagatattatatatacattttatcagtaatttttggtacattaaactcttccaagggtgaaatttaaccaaattttgtggctttgcag

SEQ ID NO: 63 - DNA, 9285 bp, synthetic construct
  source 1..9285: mol_type = other DNA
  misc_feature 1..8912: note = genomic DNA of DWF5-1
ttagtcagtacaacagatttttataattgagagaatctgagaagaggacctataccactgtggagagagtggagtaaacacagagcactaaaaatcagtgaattaaagtctacatataagtcaagattccatattgggcggagacttctgtagttccagtttttttcttcaaaaccccaaaatcagcaaaagctgaattgattgaggaagaagaagaagaagaaaaaatggtggagaacaagttggtacactctccattaatcacttatggatcaatgctcagtcttctatctttcacaccaccttttgtaatcctcatgtaagtccaacacccacttttcatattgatctatttttgttgattttattgtcttttcttgttttggggtttttgttttcttgtgtaaaagttcagatctttgaatgggttgttgtatcatgagttaaagattggatcttttttttttttttttgtttagttttggtttgatttgcttgctatagtttaactgtcttctagttataaaaatgttttttttttggtgtaattgagattcattattatttagctctaaagaagcaagtgttttctagttataaaaatgtttgttttttgggtgtaattgagattcattattatttagctctaaagaagcaagtgtttggttagagttatgcttgtatttgtttgctaactaaacatggtaatacttgtgcatgatttaatacctgtgccccctttttgatttgggaggtctaaaagagagacactagagtggatgaagtttttcttttgaaggggatgaaaagtagaaataggaataacaggttgctccaataagtgtagattctaattttagctaatatcaattgatgatggactacgtttcaatcccgaatgagtttgattcggttaaataaagcacatgcatctgttatgctccaccttttaagttttcaaaggattcacaatcaatagactattttttactagtagtctacctactgcagccccatcttttatggggttatggtacacatttgctgagtcataattttagttagtatgatcttgaaatgtggttctgtggttctttccgtagacattcgttaattggcctatacagaaaatgatttgcatttagtcatgtgaaaggagtaaaaatgctatgtaaataaaaaattacaaattgatcctgctgtaaattttttgaatgtttcaccagtaacagatgatttctgctgccttagccacagatctttccactgtgttatgtacagtagctcaaaagtgtcttgatgaggaaatgtaattgtataactgcactaatttttggaccttaatgggcctacttgcaggtggtatacaaatgtgcacgctgatgggtctatcttgaaaacgttcaatcatctaagggaaaatggtttgcaaggattaattgatatttggccaaaacctactgcaattgctgggaagctaatcatttgttatgctctatttgaggcggcactacagcttctattgcctggtaaaacagtcgaaggcccaatatctccaactggacataggcctgtctataaggtatatggcagttatgctatacacaagtacagtgtgcatcttgcatttatagtttgtgtaatttgtcttagttgagtttatttcaagtgatgcaatggttgatgtgctatgatctgtctttcctctgttcattgtacaactgtataacttgcctcttatatcctctacttattgcaggctaatggcatggcagcatatgcagtgacactgatcacatatatcagtctctggtggtagggatttcatcaatttttgctttttgactagcttgctgaatcttgagacctcgattctttatgtattggttcgttaatctcacttgccagcttcagcttgacaatgcttgggacagcattggggtcttggggacatgaatttcatcaagggaatctaaaaaaaatatgctcttttgtgtttagggcttcaacaatttgtattaaactgataaaaagttttttcacctaaacaaacaccaatcaattcgtccaaatattaatggacactaaagaatacaacaaaaataatgaattggtgcacttttaaggtcaacgtacactctatcctccccagacccttgtgttattgctattgttgttgttgttttgtatagtgtatttattgatattgtgtgactgtctctttcaaaagtttgtagagatggcatacttgtatttacttaatatgtcttcaactcgcttcctagcaggtctagttttttccatgggccaaacacatgaatttgttttatgatgggtggttgtaagacttgaatccaaaacctttgcttgctctaataccgtatccaaaaaaaataaaataaaccttaggcctaaataaaccgaaagttagcatatttaaggaatatccaagataatataaggagataacatcacattgtctcaacgtatatgagacactctaacaactcctgacgtccagaacctttacttgtttgattgttcattttatctatgagctattgtttgtgagaaaggtgcatattatggtccattaaactcatcagttcactctctctagttatgtttttttttccgtgtctttcaggtttggaatatttaatcctgcaattgtttatgaccatctgggcgagattttctctacacttatttttgggagtttagtcttctgtgttttattgtacattaaagtaagtattttaagtaccctcagtacacctcttatctctgattctttgcttagtattatacctgtctgacaccttgtgctgacatttataatttataagggtcatgttgcaccatcttccactgattccggctcatcagggaacataatagttgacttctattgggtaagcatcttttgaaaatttaactgtgaacttcactacttcattttgtgtctttataggaaaaataagcatgatgatgttataccacaaattaagtcaaggaagtcaatatctagtacttgcatcatctctggagttgaaagtgatgtcataatttatgacctgatgaactctttcagggtatggagctttatcctcgtatcgggaaacacttcgatattaaagtcttcacaaactgcagatttggtatgatgtcttgggcagttcttgctgtcacgtattgcataaaacaggtaaatgatgtaatgaagtccttgatagtgagaattaaaactttcccaatatttctcggtcctattgttcctgagttggtgaattttacaagcccttttattggggatcccttgccagttgttcagtttttaggtcatgcaagtaagaaaatgatataatattcatttgcttccgtcaatagatgtttaacaggataagaaaaagacattttcttataccatttaatggaaaaaaacagtggactgttatctaaagtactccctccgttccaatttatttgaccaattttgacttggcatggagtttaagaaagtaaagaagacttgaattttgtggtcttaaactaaaggtatgtcaaatgtaccaaaaatgcctcggggtcttaaacatgccatgtggaaagttgaaattaagagttgctaaaaaaagaaagaatcattctttttgaaatggactaaaaaggaaagcaggccaaacaaattgagaaggagggagtaattatgtttacttgacatgaccctatcacagcttaggtgtctttactttgtgctcgttctttcaccttgacccctaacattctttacctggatttcagttgattgtcaatagaaaaacctagtatatgaacttcattttgatgtttgacagtcgatagtttgtataacatattcttacttttcagcatgaagaatatgggcgtgtatctgattccatgcttgtaaatacgatattgatgttggtgtatgtcacaaaattcttttggtgggaagctgggtactggaacacaatggatattgcacatgacagaggtttgtgcatactgtgttttctatattgatatagcaagtaccttcccagtgctctgattgcaaatgctgacatttcttgtttctctatttcggtggacgcctatatataatcttctctggatctcaaattcgtttggcagctggcttttatatatgttggggatgcttggtgtgggttccaagcatatatacgtctcctggaatgtatcttgttaaacaacctgtgaatcttgggcttcaggtatttttgcatccaagaagaatttgctaaatgcatataaaatataaagttattgccaataagcattacttactgtttatttttatactcaactactattttgggatttgtacttagtttttacttagtcttcgtcttctatttgataaccaagaaatccccgagggctggtggggtacagttcgaagctcaatggataataagctcattcctcttcccttctccacttaattaccaggctattgtctgtggcaagtttctaatatatggcaaatacatatctgcagcctgcatatcatgtgcttggtcttcatctttatcaacttatttgaagaaatgttcttagtgaaccatattcacctctagttcatgcactgaaatactcaatcacgagtcacggcccacaatgtggttataatcagtgctatttatccagcttgtgagatcagatcgactactctactaccatcattccattgcctagcacgaaaggttgcttaggacaaattatggaaaatgttctttgcagtaataccaagaaagtagtagctcactgtgaaagtttcactcaaataatgttgctgaaggtgaaaggttcaaaaaaggcatcatatttctgctgaactgaaatctcctcacagtctggctttgtaacttttgtagacatataattgtaattcaaaaacacttttaaatcgaatgaacttaaggcaataatgaagagtgaaaatgagggtgactgttgagcatatggtagagagtacaaaccatgatagataacagaagatagatatcttccaaactccctgatagagtcagaagttgtggattattagtttcaagcttgagaaaacccctggagatgtgaaataatgtacttagaatatcttccaatcgacatttatccctttaaagtatgacggaagtcccattgctggcagaatcatctgtagcataacagataatatgagcaaatgagaccattcagccattcatcaatggctaacgtgttcatttttcgccaagctagcatttcttttgttgcatggatgtgtaatttttctcctttgtttcattttctttgacattttcacttttcagggtgtccattactctcttcaacattggctttattgcttcctctgttctaattgatatgacactcttttcactatgaagttgtcagatattttccaccagtctaacagtatttctcaatgactattgcttaacctcttaaaaataactgtggtttttctcgactatactattttttcgattggtttgacaatactatttactcttttgatcattcctttgatattttattcgattagcactataggtatggaaaaattaaaatactacattcaaatgtcatataaaattagaggaaaggagtatataagtttttagtcaaagagttggtaatttgtataattttatttaaaatgataatgttcgatattagaacattgagtcaaccttcttaagaggaagtacaatctgggttcgttagagtacttcagatgagttgcatcctatattttcgatgatatcttccatttctggtattttaaacgatcatgtaaagaaaaaacagaacacattcttgaattgtcaaatgaccaagaaaggttctgtattgagtgttcacttttaccaatagggtctacccttgggatgatggtgtttcacttttaaattccctgagaattgcgaccttttgcccccacccaacacaccttaggacattttagatcagtgtatgtagaatttacctgtccctattggtagcaacatacgttttacggttagaaatttgactatccaatgttatagtttcttatttgccatcagggcatgtgatattttgaaacttccgttacttcaatccactataaaaaaactacacgtattaacatggcttgtagagcgcacacattcatttgctaatagcgacataagtatctgaaaaggagagaattatgagtacaattacttccctaatgtttcatccaacttattgaccttcactagattttacaacttggatggtggatgtacttcatagtacatacggattgtttcgttagttttcacatgtttcatttgatgtattataaatgttctgcataacagaaaaacaagacttattctagaattgtctgatgaagcagagaaaggttgctgattttttttgtcaactaggggtcttcccttggggacaatggtctttcacgtgatctctctgagaattgcaatgatttgcgacgatgcaccagtttgccattttgtcattgcaaggcaaatttttggctagaaaacattgagtgataatgtgttatctgaaattgatcattggtgcattgcatcaacctgcttaaggaaaccacatgtagtaaaatgacttggagagcatatgcaattttattgctttcggtttctaacgaggaaagttctttctgttatttcagctttccctttacatactagtggctggtcttctctgcatatatatcaactatgattgtgacaggcagaggcaagagttccggagaacaaatggaaaatgcactgtctggggaaagactccatctaaggtcaaatgataccatctgtgaatttatttttcgaactctcttacccttatttgatgatttttgacttggttccttcactcaatgcagatagtcgccgcatacactactacctctggtgagaaaaagaccagccttctgcttacatcaggatggtcagttcctttctttgttctcctgctgacgttttacttctgcaatttagacactacaacagtttttttggggggaggtaataattgtatcaaattcagcactaagaaagtgctgcagaagtatatccatcagtagtcaaatccagcagttaagaatgtattctaatcctagtcttgtagggattctataagatctaaaactgttcatcatctttcattattctttgcaccaaaaaacaaaataacaaactacagatcattttgatctttttggatggaacttggtttgccttcaaaacatcttttccttcctctcccaattgtccaccaaacgcaagcaaggatggcatttcaccattttgtttggctttattcgtgcctgatttattccagctacttagtagatcattgtgattgctaggcatcatccattgaagtcccactatgtttaggaataaatgccatagctgattagtcatttgacagtgcaaaaatagatagtaatagtttctgacctttctccacacaaaaaacattttgtacaaaagtataatgcccctcttctgttaagttctcttgagtttgacttgcttccatagtcatcaagtcagtcaccatgtgaaacatgcaactttgtatggagtttttttctccatatcttcttccacggccagcacctgttccgttgagcattaatcatcagtcttgtagcatgagtagaccgtaaaggaagcaatgcttgtggcatccatattgctctttcttcataactggacagttctggagcatgctctaatgcatcaatcaatcaactattctagttagttctcagtcatttagcttactcctaaattgtgtactggattgtaaaactacgaaattgtattgttattctcctatattaccagtctcattcttatagaggctgtacttgattgcattaacaaggaattctgaataaataccttctatatttctaagaaaagcatctagaatttattctacttttcttatatcccgttttctaacgccaaacaaattcatatattgatgtataatacatgtcaattattttgcttatagcggcttgagacatcatacaatttacataatatgtttaaaccattttgcaggtggggcttagctcgccatttccactatgttccagaaatattagcggcatttttctggagtgtaccagctcttttcaaccacgtaagcgttcatttacatcattactctgtatttttcttctttccgtattagagagaattccataatcaattttatctttcttgaattttgcattttgttcttgacattgctgaaatctaacatcctgtcccccttctttactttttcttgtacttgcagttcattccctacttctacgtcatctttctaataatcctccttctcgatcgagctaaaagggacgatgaccgatgcaaggcaaagtaagaaagcacacaccctcatttttacctggatttttcatatggttctccactcctcactaataaactcgatcaaattgattagtaatagtcatacatgtcttgctggttgtgttgttaacaagacttgagaacttatcgatttctttgctcatggacagaataaacttatgatatcctcaaaataattatcctggcattccgccacccccatggcataatagatccctagaggtggcacctgagggtgtgacctagacgtcaatgaaatgattgacaatcatgggattaggggttcaaatcccaatcgaagacaaaaacttaggtgatttttaccccatttgcctagaccttaacaggcagagtagtcagtatatgtgttggtaggagttaacacgtagcaggtagagtgtagctgaaatggacgaaagctggcctagacaccactgttttttagaaaaaactagttgagtagccgaaggtcgtcttgatctgtccctaaagatcgttacgaagatattatatatacattttatcagtaatttttggtacattaaactcttccaagggtgaaatttaaccaaattttgtggctttgcaggtatggcaagtactggaaattgtattgtgaaaaggttccttacagagttatcccaggaatttactagtgatttttggacttctaagaatgttttactataaagtttgatgtattttgtagcctcttcatgttgttgtttgtatgtacacttattagttccaacagttttgagaaacttgtttttatataaaaatagtgaagacgcgagttgag

SEQ ID NO: 64 - DNA, 227 bp, synthetic construct
  source 1..227: mol_type = other DNA
  misc_feature 1..227: note = 5'UTR of DWF5-1
ttagtcagtacaacagatttttataattgagagaatctgagaagaggacctataccactgtggagagagtggagtaaacacagagcactaaaaatcagtgaattaaagtctacatataagtcaagattccatattgggcggagacttctgtagttccagtttttttcttcaaaaccccaaaatcagcaaaagctgaattgattgaggaagaagaagaagaagaaaaa

SEQ ID NO: 65 - DNA, 146 bp, synthetic construct
  source 1..146: mol_type = other DNA
  misc_feature 1..146: note = 3'UTR of DWF5-1
tgatttttggacttctaagaatgttttactataaagtttgatgtattttgtagcctcttcatgttgttgtttgtatgtacacttattagttccaacagttttgagaaacttgtttttatataaaaatagtgaagacgcgagttgag

SEQ ID NO: 66 - DNA, 88 bp, synthetic construct
  source 1..88: mol_type = other DNA
  misc_feature 1..88: note = wild type
ggtatggagctttatcctcgtatcgggaaacacttcgatattaaagtcttcacaaactgcagatttggtatgatgtcttgggcagttc

SEQ ID NO: 67 - DNA, 85 bp, synthetic construct
  source 1..85: mol_type = other DNA
  misc_feature 1..85: note = #3-11
ggtatggagctttatcctcatcgggaaacacttcgatattaaagtcttcacaaactgcagatttggtatgattcttgggcagttc

SEQ ID NO: 68 - DNA, 85 bp, synthetic construct; identical to SEQ ID NO: 67
  source 1..85: mol_type = other DNA
  misc_feature 1..85: note = #3-14

SEQ ID NO: 69 - DNA, 85 bp, synthetic construct; identical to SEQ ID NO: 67
  source 1..85: mol_type = other DNA
  misc_feature 1..85: note = #4-8

SEQ ID NO: 70 - DNA, 85 bp, synthetic construct
  source 1..85: mol_type = other DNA
  misc_feature 1..85: note = #1-4
ggtatggagctttatcctcgtaatcgggaaacacttcgatattaaagtcttcacaaactgcagatttggtattcttgggcagttc

SEQ ID NO: 71 - DNA, 85 bp, synthetic construct; identical to SEQ ID NO: 70
  source 1..85: mol_type = other DNA
  misc_feature 1..85: note = #7-1

SEQ ID NO: 72 - DNA, 85 bp, synthetic construct; identical to SEQ ID NO: 70
  source 1..85: mol_type = other DNA
  misc_feature 1..85: note = #12-8

SEQ ID NO: 73 - DNA, 269 bp, synthetic construct
  source 1..269: mol_type = other DNA
  misc_feature 1..269: note = wild type
atggagctttatcctcgtatcgggaaacacttcgatattaaagtcttcacaaactgcagatttggtatgatgtcttgggcagttcttgctgtcacgtattgcataaaacagcatgaagaatatgggcgtgtatctgattccatgcttgtaaatacgatattgatgttggtgtatgtcacaaaattcttttggtgggaagctgggtactggaacacaatggatattgcacatgacagagctggcttttatatatgttggggatgcttggt

SEQ ID NO: 74 - DNA, 266 bp, synthetic construct
  source 1..266: mol_type = other DNA
  misc_feature 1..266: note = D100_3-14-29
atggagctttatcctcatcgggaaacacttcgatattaaagtcttcacaaactgcagatttggtatgattcttgggcagttcttgctgtcacgtattgcataaaacagcatgaagaatatgggcgtgtatctgattccatgcttgtaaatacgatattgatgttggtgtatgtcacaaaattcttttggtgggaagctgggtactggaacacaatggatattgcacatgacagagctggcttttatatatgttggggatgcttggt

SEQ ID NO: 75 - DNA, 266 bp, synthetic construct
  source 1..266: mol_type = other DNA
  misc_feature 1..266: note = D100_7-1-15
atggagctttatcctcgtaatcgggaaacacttcgatattaaagtcttcacaaactgcagatttggtattcttgggcagttcttgctgtcacgtattgcataaaacagcatgaagaatatgggcgtgtatctgattccatgcttgtaaatacgatattgatgttggtgtatgtcacaaaattcttttggtgggaagctgggtactggaacacaatggatattgcacatgacagagctggcttttatatatgttggggatgcttggt

SEQ ID NO: 76 - protein, 89 aa, synthetic construct
  REGION 1..89: note = wild type
MELYPRIGKHFDIKVFTNCRFGMMSWAVLAVTYCIKQHEEYGRVSDSMLVNTILMLVYVTKFFWWEAGYWNTMDIAHDRAGFYICWGCL

SEQ ID NO: 77 - protein, 88 aa, synthetic construct
  REGION 1..88: note = D100_3-14-29
MELYPHRETLRYXSLHKLQIWYDSWAVLAVTYCIKQHEEYGRVSDSMLVNTILMLVYVTKFFWWEAGYWNTMDIAHDRAGFYICWGCL

SEQ ID NO: 78 - protein, 88 aa, synthetic construct
  REGION 1..88: note = D100_7-1-15
MELYPRNRETLRYXSLHKLQIWYSWAVLAVTYCIKQHEEYGRVSDSMLVNTILMLVYVTKFFWWEAGYWNTMDIAHDRAGFYICWGCL